European Patent Specification EP 4 127 247 B1, published July 8, 2026. Title: Assays for the Detection of SARS-CoV-2. Applicant: DiaSorin S.p.A. Brambati, Chiara Bocchetta, Simone Minnucci, Giulia. The sequence listing filed with the application follows.

SEQUENCE LISTING (415 sequences)

SEQ ID NO: 1 - DNA, 20 bp, SARS-CoV-2 Coronavirus
  misc_feature (1)..(20): Preferred Forward ORF1ab Gene Primer
atggtagagttgatggtcaa

SEQ ID NO: 2 - DNA, 20 bp, SARS-CoV2 Coronavirus
  misc_feature (1)..(20): Preferred Reverse ORF1ab Gene Primer
taagactagcttgtttggga

SEQ ID NO: 3 - DNA, 117 bp, SARS-CoV2 Coronavirus
  misc_feature (1)..(117): Amplified Region of ORF1ab Gene ("Sense" Strand)
atggtagagttgatggtcaagtagacttatttagaaatgcccgtaatggtgttcttattacagaaggtagtgttaaaggtttacaaccatctgtaggtcccaaacaagctagtctta

SEQ ID NO: 4 - DNA, 117 bp, SARS-CoV2 Coronavirus
  misc_feature (1)..(117): Amplified Region of ORF1ab Gene ("Anti-Sense" Strand)
taagactagcttgtttgggacctacagatggttgtaaacctttaacactaccttctgtaataagaacaccattacgggcatttctaaataagtctacttgaccatcaactctaccat

SEQ ID NO: 5 - DNA, 20 bp, SARS-CoV2 Coronavirus
  misc_feature (1)..(20): Preferred Forward S Gene Primer
ctaaccaggttgctgttctt

SEQ ID NO: 6 - DNA, 20 bp, SARS-CoV2 Coronavirus
  misc_feature (1)..(20): Preferred Reverse S Gene Primer
cctgtagaataaacacgcca

SEQ ID NO: 7 - DNA, 103 bp, SARS-CoV2 Coronavirus
  misc_feature (1)..(103): Amplified Region of S Gene ("Sense" Strand)
ctaaccaggttgctgttctttatcaggatgttaactgcacagaagtccctgttgctattcatgcagatcaacttactcctacttggcgtgtttattctacagg

SEQ ID NO: 8 - DNA, 103 bp, SARS-CoV2 Coronavirus
  misc_feature (1)..(103): Amplified Region of S Gene ("Anti-Sernse" Strand)
cctgtagaataaacacgccaagtaggagtaagttgatctgcatgaatagcaacagggacttctgtgcagttaacatcctgataaagaacagcaacctggttag

SEQ ID NO: 9 - DNA, 27 bp, SARS-CoV2 Coronavirus
  misc_feature (1)..(27): Preferred ORF1ab Gene Probe
tgcccgtaatggtgttcttattacaga

SEQ ID NO: 10 - DNA, 27 bp, SARS-CoV2 Coronavirus
  misc_feature (1)..(27): Preferred Complement ORF1ab Probe
tctgtaataagaacaccattacgggca

SEQ ID NO: 11 - DNA, 21 bp, SARS-CoV2 Coronavirus
  misc_feature (1)..(21): Preferred S Gene Probe
tgcacagaagtccctgttgct

SEQ ID NO: 12 - DNA, 21 bp, SARS-CoV2 Coronavirus
  misc_feature (1)..(21): Preferred Complement S Gene Probe
agcaacagggacttctgtgca

SEQ ID NO: 13 - DNA, 16 bp, Bacteriophage MS2
  misc_feature (1)..(16): Forward MS2 Phage Internal Control Primer
tgctcgcggatacccg

SEQ ID NO: 14 - DNA, 20 bp, Bacteriophage MS2
  misc_feature (1)..(20): Reverse MS2 Phage Internal Control Primer
aacttgcgttctcgagcgat

SEQ ID NO: 15 - DNA, 24 bp, Bacteriophage MS2
  misc_feature (1)..(24): MS2 Phage Internal Control Probe
acctcgggtttccgtcttgctcgt

SEQ ID NO: 16 - DNA, 3819 bp, SARS-CoV2 Coronavirus
  misc_feature (1)..(3819): S Gene of SARS-CoV-2 of GenBank NC_045512
atgtttgtttttcttgttttattgccactagtctctagtcagtgtgttaatcttacaaccagaactcaattaccccctgcatacactaattctttcacacgtggtgtttattaccctgacaaagttttcagatcctcagttttacattcaactcaggacttgttcttacctttcttttccaatgttacttggttccatgctatacatgtctctgggaccaatggtactaagaggtttgataaccctgtcctaccatttaatgatggtgtttattttgcttccactgagaagtctaacataataagaggctggatttttggtactactttagattcgaagacccagtccctacttattgttaataacgctactaatgttgttattaaagtctgtgaatttcaattttgtaatgatccatttttgggtgtttattaccacaaaaacaacaaaagttggatggaaagtgagttcagagtttattctagtgcgaataattgcacttttgaatatgtctctcagccttttcttatggaccttgaaggaaaacagggtaatttcaaaaatcttagggaatttgtgtttaagaatattgatggttattttaaaatatattctaagcacacgcctattaatttagtgcgtgatctccctcagggtttttcggctttagaaccattggtagatttgccaataggtattaacatcactaggtttcaaactttacttgctttacatagaagttatttgactcctggtgattcttcttcaggttggacagctggtgctgcagcttattatgtgggttatcttcaacctaggacttttctattaaaatataatgaaaatggaaccattacagatgctgtagactgtgcacttgaccctctctcagaaacaaagtgtacgttgaaatccttcactgtagaaaaaggaatctatcaaacttctaactttagagtccaaccaacagaatctattgttagatttcctaatattacaaacttgtgcccttttggtgaagtttttaacgccaccagatttgcatctgtttatgcttggaacaggaagagaatcagcaactgtgttgctgattattctgtcctatataattccgcatcattttccacttttaagtgttatggagtgtctcctactaaattaaatgatctctgctttactaatgtctatgcagattcatttgtaattagaggtgatgaagtcagacaaatcgctccagggcaaactggaaagattgctgattataattataaattaccagatgattttacaggctgcgttatagcttggaattctaacaatcttgattctaaggttggtggtaattataattacctgtatagattgtttaggaagtctaatctcaaaccttttgagagagatatttcaactgaaatctatcaggccggtagcacaccttgtaatggtgttgaaggttttaattgttactttcctttacaatcatatggtttccaacccactaatggtgttggttaccaaccatacagagtagtagtactttcttttgaacttctacatgcaccagcaactgtttgtggacctaaaaagtctactaatttggttaaaaacaaatgtgtcaatttcaacttcaatggtttaacaggcacaggtgttcttactgagtctaacaaaaagtttctgcctttccaacaatttggcagagacattgctgacactactgatgctgtccgtgatccacagacacttgagattcttgacattacaccatgttcttttggtggtgtcagtgttataacaccaggaacaaatacttctaaccaggttgctgttctttatcaggatgttaactgcacagaagtccctgttgctattcatgcagatcaacttactcctacttggcgtgtttattctacaggttctaatgtttttcaaacacgtgcaggctgtttaataggggctgaacatgtcaacaactcatatgagtgtgacatacccattggtgcaggtatatgcgctagttatcagactcagactaattctcctcggcgggcacgtagtgtagctagtcaatccatcattgcctacactatgtcacttggtgcagaaaattcagttgcttactctaataactctattgccatacccacaaattttactattagtgttaccacagaaattctaccagtgtctatgaccaagacatcagtagattgtacaatgtacatttgtggtgattcaactgaatgcagcaatcttttgttgcaatatggcagtttttgtacacaattaaaccgtgctttaactggaatagctgttgaacaagacaaaaacacccaagaagtttttgcacaagtcaaacaaatttacaaaacaccaccaattaaagattttggtggttttaatttttcacaaatattaccagatccatcaaaaccaagcaagaggtcatttattgaagatctacttttcaacaaagtgacacttgcagatgctggcttcatcaaacaatatggtgattgccttggtgatattgctgctagagacctcatttgtgcacaaaagtttaacggccttactgttttgccacctttgctcacagatgaaatgattgctcaatacacttctgcactgttagcgggtacaatcacttctggttggacctttggtgcaggtgctgcattacaaataccatttgctatgcaaatggcttataggtttaatggtattggagttacacagaatgttctctatgagaaccaaaaattgattgccaaccaatttaatagtgctattggcaaaattcaagactcactttcttccacagcaagtgcacttggaaaacttcaagatgtggtcaaccaaaatgcacaagctttaaacacgcttgttaaacaacttagctccaattttggtgcaatttcaagtgttttaaatgatatcctttcacgtcttgacaaagttgaggctgaagtgcaaattgataggttgatcacaggcagacttcaaagtttgcagacatatgtgactcaacaattaattagagctgcagaaatcagagcttctgctaatcttgctgctactaaaatgtcagagtgtgtacttggacaatcaaaaagagttgatttttgtggaaagggctatcatcttatgtccttccctcagtcagcacctcatggtgtagtcttcttgcatgtgacttatgtccctgcacaagaaaagaacttcacaactgctcctgccatttgtcatgatggaaaagcacactttcctcgtgaaggtgtctttgtttcaaatggcacacactggtttgtaacacaaaggaatttttatgaaccacaaatcattactacagacaacacatttgtgtctggtaactgtgatgttgtaataggaattgtcaacaacacagtttatgatcctttgcaacctgaattagactcattcaaggaggagttagataaatattttaagaatcatacatcaccagatgttgatttaggtgacatctctggcattaatgcttcagttgtaaacattcaaaaagaaattgaccgcctcaatgaggttgccaagaatttaaatgaatctctcatcgatctccaagaacttggaaagtatgagcagtatataaaatggccatggtacatttggctaggttttatagctggcttgattgccatagtaatggtgacaattatgctttgctgtatgaccagttgctgtagttgtctcaagggctgttgttcttgtggatcctgctgcaaatttgatgaagacgactctgagccagtgctcaaaggagtcaaattacattacaca

SEQ ID NO: 17 - DNA, 19 bp, SARS-CoV2 Coronavirus
  misc_feature (1)..(19): Illustrative Variant Forward ORF1ab Primer
atggtagagttgatggtca

SEQ ID NO: 18 - DNA, 18 bp, SARS-CoV2 Coronavirus
  misc_feature (1)..(18): Illustrative Variant Forward ORF1ab Primer
atggtagagttgatggtc

SEQ ID NO: 19 - DNA, 17 bp, SARS-CoV2 Coronavirus
  misc_feature (1)..(17): Illustrative Variant Forward ORF1ab Primer
atggtagagttgatggt

SEQ ID NO: 20 - DNA, 16 bp, SARS-CoV2 Coronavirus
  misc_feature (1)..(16): Illustrative Variant Forward ORF1ab Primer
atggtagagttgatgg

SEQ ID NO: 21 - DNA, 15 bp, SARS-CoV2 Coronavirus
  misc_feature (1)..(15): Illustrative Variant Forward ORF1ab Primer
atggtagagttgatg

SEQ ID NO: 22 - DNA, 19 bp, SARS-CoV2 Coronavirus
  misc_feature (1)..(19): Illustrative Variant Forward ORF1ab Primer
tggtagagttgatggtcaa

SEQ ID NO: 23 - DNA, 18 bp, SARS-CoV2 Coronavirus
  misc_feature (1)..(18): Illustrative Variant Forward ORF1ab Primer
ggtagagttgatggtcaa

SEQ ID NO: 24 - DNA, 17 bp, SARS-CoV2 Coronavirus
  misc_feature (1)..(17): Illustrative Variant Forward ORF1ab Primer
gtagagttgatggtcaa

SEQ ID NO: 25 - DNA, 16 bp, SARS-CoV2 Coronavirus
  misc_feature (1)..(16): Illustrative Variant Forward ORF1ab Primer
tagagttgatggtcaa

SEQ ID NO: 26 - DNA, 15 bp, SARS-CoV2 Coronavirus
  misc_feature (1)..(15): Illustrative Variant Forward ORF1ab Primer
agagttgatggtcaa

SEQ ID NO: 27 - DNA, 18 bp, SARS-CoV2 Coronavirus
  misc_feature (1)..(18): Illustrative Variant Forward ORF1ab Primer
tggtagagttgatggtca

SEQ ID NO: 28 - DNA, 16 bp, SARS-CoV2 Coronavirus
  misc_feature (1)..(16): Illustrative Variant Forward ORF1ab Primer
ggtagagttgatggtc

SEQ ID NO: 29 - DNA, 19 bp, SARS-CoV2 Coronavirus
  misc_feature (1)..(19): Illustrative Variant Reverse ORF1ab Primer
taagactagcttgtttggg

SEQ ID NO: 30 - DNA, 18 bp, SARS-CoV2 Coronavirus
  misc_feature (1)..(19): Illustrative Variant Reverse ORF1ab Primer
taagactagcttgtttgg

SEQ ID NO: 31 - DNA, 17 bp, SARS-CoV2 Coronavirus
  misc_feature (1)..(17): Illustrative Variant Reverse ORF1ab Primer
taagactagcttgtttg

SEQ ID NO: 32 - DNA, 16 bp, SARS-CoV2 Coronavirus
  misc_feature (1)..(16): Illustrative Variant Reverse ORF1ab Primer
taagactagcttgttt

SEQ ID NO: 33 - DNA, 15 bp, SARS-CoV2 Coronavirus
  misc_feature (1)..(15): Illustrative Variant Reverse ORF1ab Primer
taagactagcttgtt

SEQ ID NO: 34 - DNA, 19 bp, SARS-CoV2 Coronavirus
  misc_feature (1)..(19): Illustrative Variant Reverse ORF1ab Primer
aagactagcttgtttggga

SEQ ID NO: 35 - DNA, 18 bp, SARS-CoV2 Coronavirus
  misc_feature (1)..(18): Illustrative Variant Reverse ORF1ab Primer
agactagcttgtttggga

SEQ ID NO: 36 - DNA, 17 bp, SARS-CoV2 Coronavirus
  misc_feature (1)..(17): Illustrative Variant Reverse ORF1ab Primer
gactagcttgtttggga

SEQ ID NO: 37 - DNA, 16 bp, SARS-CoV2 Coronavirus
  misc_feature (1)..(16): Illustrative Variant Reverse ORF1ab Primer
actagcttgtttggga

SEQ ID NO: 38 - DNA, 15 bp, SARS-CoV2 Coronavirus
  misc_feature (1)..(15): Illustrative Variant Reverse ORF1ab Primer
ctagcttgtttggga

SEQ ID NO: 39 - DNA, 18 bp, SARS-CoV2 Coronavirus
  misc_feature (1)..(18): Illustrative Variant Reverse ORF1ab Primer
aagactagcttgtttggg

SEQ ID NO: 40 - DNA, 17 bp, SARS-CoV2 Coronavirus
  misc_feature (1)..(17): Illustrative Variant Reverse ORF1ab Primer
agactagcttgtttggg

SEQ ID NO: 41 - DNA, 16 bp, SARS-CoV2 Coronavirus
  misc_feature (1)..(16): Illustrative Variant Reverse ORF1ab Primer
agactagcttgtttgg

SEQ ID NO: 42 - DNA, 15 bp, SARS-CoV2 Coronavirus
  misc_feature (1)..(15): Illustrative Variant Reverse ORF1ab Primer
gactagcttgtttgg

SEQ ID NO: 43 - DNA, 28 bp, SARS-CoV2 Coronavirus
  misc_feature (1)..(28): Illustrative Variant Forward S Gene Primer
ctaaccaggttgctgttctttatcagga

SEQ ID NO: 44 - DNA, 28 bp, SARS-CoV2 Coronavirus
  misc_feature (1)..(28): Illustrative Variant Forward S Gene Primer
ctaaccaggttgctgttctttatcaggg

SEQ ID NO: 45 - DNA, 27 bp, SARS-CoV2 Coronavirus
  misc_feature (1)..(27): Illustrative Variant Forward S Gene Primer
taaccaggttgctgttctttatcagga

SEQ ID NO: 46 - DNA, 27 bp, SARS-CoV2 Coronavirus
  misc_feature (1)..(27): Illustrative Variant Forward S Gene Primer
taaccaggttgctgttctttatcaggg

SEQ ID NO: 47 - DNA, 26 bp, SARS-CoV2 Coronavirus
  misc_feature (1)..(26): Illustrative Variant Forward S Gene Primer
aaccaggttgctgttctttatcagga

SEQ ID NO: 48 - DNA, 26 bp, SARS-CoV2 Coronavirus
  misc_feature (1)..(26): Illustrative Variant Forward S Gene Primer
aaccaggttgctgttctttatcaggg

SEQ ID NO: 49 - DNA, 25 bp, SARS-CoV2 Coronavirus
  misc_feature (1)..(25): Illustrative Variant Forward S Gene Primer
accaggttgctgttctttatcagga

SEQ ID NO: 50 - DNA, 25 bp, SARS-CoV2 Coronavirus
  misc_feature (1)..(25): Illustrative Variant Forward S Gene Primer
accaggttgctgttctttatcaggg

SEQ ID NO: 51 - DNA, 24 bp, SARS-CoV2 Coronavirus
  misc_feature (1)..(24): Illustrative Variant Forward S Gene Primer
ccaggttgctgttctttatcagga

SEQ ID NO: 52 - DNA, 24 bp, SARS-CoV2 Coronavirus
  misc_feature (1)..(24): Illustrative Variant Forward S Gene Primer
ccaggttgctgttctttatcaggg

SEQ ID NO: 53 - DNA, 23 bp, SARS-CoV2 Coronavirus
  misc_feature (1)..(23): Illustrative Variant Forward S Gene Primer
caggttgctgttctttatcagga

SEQ ID NO: 54 - DNA, 23 bp, SARS-CoV2 Coronavirus
  misc_feature (1)..(23): Illustrative Variant Forward S Gene Primer
caggttgctgttctttatcaggg

SEQ ID NO: 55 - DNA, 22 bp, SARS-CoV2 Coronavirus
  misc_feature (1)..(22): Illustrative Variant Forward S Gene Primer
aggttgctgttctttatcagga

SEQ ID NO: 56 - DNA, 22 bp, SARS-CoV2 Coronavirus
  misc_feature (1)..(22): Illustrative Variant Forward S Gene Primer
aggttgctgttctttatcaggg

SEQ ID NO: 57 - DNA, 21 bp, SARS-CoV2 Coronavirus
  misc_feature (1)..(21): Illustrative Variant Forward S Gene Primer
ggttgctgttctttatcagga

SEQ ID NO: 58 - DNA, 21 bp, SARS-CoV2 Coronavirus
  misc_feature (1)..(21): Illustrative Variant Forward S Gene Primer
ggttgctgttctttatcaggg

SEQ ID NO: 59 - DNA, 20 bp, SARS-CoV2 Coronavirus
  misc_feature (1)..(20): Illustrative Variant Forward S Gene Primer
gttgctgttctttatcagga

SEQ ID NO: 60 - DNA, 20 bp, SARS-CoV2 Coronavirus
  misc_feature (1)..(20): Illustrative Variant Forward S Gene Primer
gttgctgttctttatcaggg

SEQ ID NO: 61 - DNA, 19 bp, SARS-CoV2 Coronavirus
  misc_feature (1)..(19): Illustrative Variant Forward S Gene Primer
ttgctgttctttatcagga

SEQ ID NO: 62 - DNA, 19 bp, SARS-CoV2 Coronavirus
  misc_feature (1)..(19): Illustrative Variant Forward S Gene Primer
ttgctgttctttatcaggg

SEQ ID NO: 63 - DNA, 18 bp, SARS-CoV2 Coronavirus
  misc_feature (1)..(18): Illustrative Variant Forward S Gene Primer
tgctgttctttatcagga

SEQ ID NO: 64 - DNA, 18 bp, SARS-CoV2 Coronavirus
  misc_feature (1)..(18): Illustrative Variant Forward S Gene Primer
tgctgttctttatcaggg

SEQ ID NO: 65 - DNA, 17 bp, SARS-CoV2 Coronavirus
  misc_feature (1)..(17): Illustrative Variant Forward S Gene Primer
gctgttctttatcagga

SEQ ID NO: 66 - DNA, 17 bp, SARS-CoV2 Coronavirus
  misc_feature (1)..(17): Illustrative Variant Forward S Gene Primer
gctgttctttatcaggg

SEQ ID NO: 67 - DNA, 16 bp, SARS-CoV2 Coronavirus
  misc_feature (1)..(16): Illustrative Variant Forward S Gene Primer
ctgttctttatcagga

SEQ ID NO: 68 - DNA, 16 bp, SARS-CoV2 Coronavirus
  misc_feature (1)..(16): Illustrative Variant Forward S Gene Primer
ctgttctttatcaggg

SEQ ID NO: 69 - DNA, 15 bp, SARS-CoV2 Coronavirus
  misc_feature (1)..(15): Illustrative Variant Forward S Gene Primer
tgttctttatcagga

SEQ ID NO: 70 - DNA, 15 bp, SARS-CoV2 Coronavirus
  misc_feature (1)..(15): Illustrative Variant Forward S Gene Primer
tgttctttatcaggg

SEQ ID NO: 71 - DNA, 19 bp, SARS-CoV2 Coronavirus
  misc_feature (1)..(19): Illustrative Variant Forward S Gene Primer
ctaaccaggttgctgttct

SEQ ID NO: 72 - DNA, 18 bp, SARS-CoV2 Coronavirus
  misc_feature (1)..(18): Illustrative Variant Forward S Gene Primer
ctaaccaggttgctgttc

SEQ ID NO: 73 - DNA, 17 bp, SARS-CoV2 Coronavirus
  misc_feature (1)..(17): Illustrative Variant Forward S Gene Primer
ctaaccaggttgctgtt

SEQ ID NO: 74 - DNA, 16 bp, SARS-CoV2 Coronavirus
  misc_feature (1)..(16): Illustrative Variant Forward S Gene Primer
ctaaccaggttgctgt

SEQ ID NO: 75 - DNA, 15 bp, SARS-CoV2 Coronavirus
  misc_feature (1)..(15): Illustrative Variant Forward S Gene Primer
ctaaccaggttgctg

SEQ ID NO: 76 - DNA, 19 bp, SARS-CoV2 Coronavirus
  misc_feature (1)..(19): Illustrative Variant Forward S Gene Primer
taaccaggttgctgttctt

SEQ ID NO: 77 - DNA, 18 bp, SARS-CoV2 Coronavirus
  misc_feature (1)..(18): Illustrative Variant Forward S Gene Primer
aaccaggttgctgttctt

SEQ ID NO: 78 - DNA, 17 bp, SARS-CoV2 Coronavirus
  misc_feature (1)..(17): Illustrative Variant Forward S Gene Primer
accaggttgctgttctt

SEQ ID NO: 79 - DNA, 16 bp, SARS-CoV2 Coronavirus
  misc_feature (1)..(16): Illustrative Variant Forward S Gene Primer
ccaggttgctgttctt

SEQ ID NO: 80 - DNA, 15 bp, SARS-CoV2 Coronavirus
  misc_feature (1)..(15): Illustrative Variant Forward S Gene Primer
caggttgctgttctt

SEQ ID NO: 81 - DNA, 18 bp, SARS-CoV2 Coronavirus
  misc_feature (1)..(18): Illustrative Variant Forward S Gene Primer
taaccaggttgctgttct

SEQ ID NO: 82 - DNA, 17 bp, SARS-CoV2 Coronavirus
  misc_feature (1)..(17): Illustrative Variant Forward S Gene Primer
aaccaggttgctgttct

SEQ ID NO: 83 - DNA, 16 bp, SARS-CoV2 Coronavirus
  misc_feature (1)..(16): Illustrative Variant Forward S Gene Primer
aaccaggttgctgttc

SEQ ID NO: 84 - DNA, 15 bp, SARS-CoV2 Coronavirus
  misc_feature (1)..(15): Illustrative Variant Forward S Gene Primer
accaggttgctgttc

SEQ ID NO: 85 - DNA, 28 bp, SARS-CoV2 Coronavirus
  misc_feature (1)..(28): Illustrative Variant Reverse S Gene Primer
gcaacagggacttctgtgcagttaacat

SEQ ID NO: 86 - DNA, 28 bp, SARS-CoV2 Coronavirus
  misc_feature (1)..(28): Illustrative Variant Reverse S Gene Primer
gcaacagggacttctgtgcagttaacac

SEQ ID NO: 87 - DNA, 27 bp, SARS-CoV2 Coronavirus
  misc_feature (1)..(27): Illustrative Variant Reverse S Gene Primer
caacagggacttctgtgcagttaacat

SEQ ID NO: 88 - DNA, 27 bp, SARS-CoV2 Coronavirus
  misc_feature (1)..(27): Illustrative Variant Reverse S Gene Primer
caacagggacttctgtgcagttaacac

SEQ ID NO: 89 - DNA, 26 bp, SARS-CoV2 Coronavirus
  misc_feature (1)..(26): Illustrative Variant Reverse S Gene Primer
aacagggacttctgtgcagttaacat

SEQ ID NO: 90 - DNA, 26 bp, SARS-CoV2 Coronavirus
  misc_feature (1)..(26): Illustrative Variant Reverse S Gene Primer
aacagggacttctgtgcagttaacac

SEQ ID NO: 91 - DNA, 25 bp, SARS-CoV2 Coronavirus
  misc_feature (1)..(25): Illustrative Variant Reverse S Gene Primer
acagggacttctgtgcagttaacat

SEQ ID NO: 92 - DNA, 25 bp, SARS-CoV2 Coronavirus
  misc_feature (1)..(25): Illustrative Variant Reverse S Gene Primer
acagggacttctgtgcagttaacac

SEQ ID NO: 93 - DNA, 24 bp, SARS-CoV2 Coronavirus
  misc_feature (1)..(24): Illustrative Variant Reverse S Gene Primer
cagggacttctgtgcagttaacat

SEQ ID NO: 94 - DNA, 24 bp, SARS-CoV2 Coronavirus
  misc_feature (1)..(24): Illustrative Variant Reverse S Gene Primer
cagggacttctgtgcagttaacac

SEQ ID NO: 95 - DNA, 23 bp, SARS-CoV2 Coronavirus
  misc_feature (1)..(23): Illustrative Variant Reverse S Gene Primer
agggacttctgtgcagttaacat

SEQ ID NO: 96 - DNA, 23 bp, SARS-CoV2 Coronavirus
  misc_feature (1)..(23): Illustrative Variant Reverse S Gene Primer
agggacttctgtgcagttaacac

SEQ ID NO: 97 - DNA, 22 bp, SARS-CoV2 Coronavirus
  misc_feature (1)..(22): Illustrative Variant Reverse S Gene Primer
gggacttctgtgcagttaacat

SEQ ID NO: 98 - DNA, 22 bp, SARS-CoV2 Coronavirus
  misc_feature (1)..(22): Illustrative Variant Reverse S Gene Primer
gggacttctgtgcagttaacac

SEQ ID NO: 99 - DNA, 21 bp, SARS-CoV2 Coronavirus
  misc_feature (1)..(21): Illustrative Variant Reverse S Gene Primer
ggacttctgtgcagttaacat

SEQ ID NO: 100 - DNA, 21 bp, SARS-CoV2 Coronavirus
  misc_feature (1)..(21): Illustrative Variant Reverse S Gene Primer
ggacttctgtgcagttaacac

SEQ ID NO: 101 - DNA, 20 bp, SARS-CoV2 Coronavirus
  misc_feature (1)..(20): Illustrative Variant Reverse S Gene Primer
gacttctgtgcagttaacat

SEQ ID NO: 102 - DNA, 20 bp, SARS-CoV2 Coronavirus
  misc_feature (1)..(20): Illustrative Variant Reverse S Gene Primer
gacttctgtgcagttaacac

SEQ ID NO: 103 - DNA, 19 bp, SARS-CoV2 Coronavirus
  misc_feature (1)..(19): Illustrative Variant Reverse S Gene Primer
acttctgtgcagttaacat

SEQ ID NO: 104 - DNA, 19 bp, SARS-CoV2 Coronavirus
  misc_feature (1)..(19): Illustrative Variant Reverse S Gene Primer
acttctgtgcagttaacac

SEQ ID NO: 105 - DNA, 18 bp, SARS-CoV2 Coronavirus
  misc_feature (1)..(18): Illustrative Variant Reverse S Gene Primer
cttctgtgcagttaacat

SEQ ID NO: 106 - DNA, 18 bp, SARS-CoV2 Coronavirus
  misc_feature (1)..(18): Illustrative Variant Reverse S Gene Primer
cttctgtgcagttaacac

SEQ ID NO: 107 - DNA, 17 bp, SARS-CoV2 Coronavirus
  misc_feature (1)..(17): Illustrative Variant Reverse S Gene Primer
ttctgtgcagttaacat

SEQ ID NO: 108 - DNA, 17 bp, SARS-CoV2 Coronavirus
  misc_feature (1)..(17): Illustrative Variant Reverse S Gene Primer
ttctgtgcagttaacac

SEQ ID NO: 109 - DNA, 16 bp, SARS-CoV2 Coronavirus
  misc_feature (1)..(16): Illustrative Variant Reverse S Gene Primer
tctgtgcagttaacat

SEQ ID NO: 110 - DNA, 16 bp, SARS-CoV2 Coronavirus
  misc_feature (1)..(16): Illustrative Variant Reverse S Gene Primer
tctgtgcagttaacac

SEQ ID NO: 111 - DNA, 15 bp, SARS-CoV2 Coronavirus
  misc_feature (1)..(15): Illustrative Variant Reverse S Gene Primer
ctgtgcagttaacat

SEQ ID NO: 112 - DNA, 15 bp, SARS-CoV2 Coronavirus
  misc_feature (1)..(15): Illustrative Variant Reverse S Gene Primer
ctgtgcagttaacac

SEQ ID NO: 113 - DNA, 19 bp, SARS-CoV2 Coronavirus
  misc_feature (1)..(19): Illustrative Variant Reverse S Gene Primer
cctgtagaataaacacgcc

SEQ ID NO: 114 - DNA, 18 bp, SARS-CoV2 Coronavirus
  misc_feature (1)..(18): Illustrative Variant Reverse S Gene Primer
cctgtagaataaacacgc

SEQ ID NO: 115 - DNA, 17 bp, SARS-CoV2 Coronavirus
  misc_feature (1)..(17): Illustrative Variant Reverse S Gene Primer
cctgtagaataaacacg

SEQ ID NO: 116 - DNA, 16 bp, SARS-CoV2 Coronavirus
  misc_feature (1)..(16): Illustrative Variant Reverse S Gene Primer
cctgtagaataaacac

SEQ ID NO: 117 - DNA, 15 bp, SARS-CoV2 Coronavirus
  misc_feature (1)..(15): Illustrative Variant Reverse S Gene Primer
cctgtagaataaaca

SEQ ID NO: 118 - DNA, 19 bp, SARS-CoV2 Coronavirus
  misc_feature (1)..(19): Illustrative Variant Reverse S Gene Primer
ctgtagaataaacacgcca

SEQ ID NO: 119 - DNA, 18 bp, SARS-CoV2 Coronavirus
  misc_feature (1)..(18): Illustrative Variant Reverse S Gene Primer
tgtagaataaacacgcca

SEQ ID NO: 120 - DNA, 17 bp, SARS-CoV2 Coronavirus
  misc_feature (1)..(17): Illustrative Variant Reverse S Gene Primer
gtagaataaacacgcca

SEQ ID NO: 121 - DNA, 16 bp, SARS-CoV2 Coronavirus
  misc_feature (1)..(16): Illustrative Variant Reverse S Gene Primer
tagaataaacacgcca

SEQ ID NO: 122 - DNA, 15 bp, SARS-CoV2 Coronavirus
  misc_feature (1)..(15): Illustrative Variant Reverse S Gene Primer
agaataaacacgcca

SEQ ID NO: 123 - DNA, 18 bp, SARS-CoV2 Coronavirus
  misc_feature (1)..(18): Illustrative Variant Reverse S Gene Primer
ctgtagaataaacacgcc

SEQ ID NO: 124 - DNA, 17 bp, SARS-CoV2 Coronavirus
  misc_feature (1)..(17): Illustrative Variant Reverse S Gene Primer
tgtagaataaacacgcc

SEQ ID NO: 125 - DNA, 16 bp, SARS-CoV2 Coronavirus
  misc_feature (1)..(16): Illustrative Variant Reverse S Gene Primer
tgtagaataaacacgc

SEQ ID NO: 126 - DNA, 15 bp, SARS-CoV2 Coronavirus
  misc_feature (1)..(15): Illustrative Variant Reverse S Gene Primer
gtagaataaacacgc

SEQ ID NO: 127 - DNA, 26 bp, SARS-CoV2 Coronavirus
  misc_feature (1)..(26): SARS-CoV-2 Polynucleotide Domain of Illustrative Sense-Strand Probe for Detecting SARS-CoV-2 ORF1ab
tgcccgtaatggtgttcttattacag

SEQ ID NO: 128 - DNA, 25 bp, SARS-CoV2 Coronavirus
  misc_feature (1)..(25): SARS-CoV-2 Polynucleotide Domain of Illustrative Sense-Strand Probe for Detecting SARS-CoV-2 ORF1ab
tgcccgtaatggtgttcttattaca

SEQ ID NO: 129 - DNA, 24 bp, SARS-CoV2 Coronavirus
  misc_feature (1)..(24): SARS-CoV-2 Polynucleotide Domain of Illustrative Sense-Strand Probe for Detecting SARS-CoV-2 ORF1ab
tgcccgtaatggtgttcttattac

SEQ ID NO: 130 - DNA, 23 bp, SARS-CoV2 Coronavirus
  misc_feature (1)..(23): SARS-CoV-2 Polynucleotide Domain of Illustrative Sense-Strand Probe for Detecting SARS-CoV-2 ORF1ab
tgcccgtaatggtgttcttatta

SEQ ID NO: 131 - DNA, 22 bp, SARS-CoV2 Coronavirus
  misc_feature (1)..(22): SARS-CoV-2 Polynucleotide Domain of Illustrative Sense-Strand Probe for Detecting SARS-CoV-2 ORF1ab
tgcccgtaatggtgttcttatt

SEQ ID NO: 132 - DNA, 21 bp, SARS-CoV2 Coronavirus
  misc_feature (1)..(21): SARS-CoV-2 Polynucleotide Domain of Illustrative Sense-Strand Probe for Detecting SARS-CoV-2 ORF1ab
tgcccgtaatggtgttcttat

SEQ ID NO: 133 - DNA, 20 bp, SARS-CoV2 Coronavirus
  misc_feature (1)..(20): SARS-CoV-2 Polynucleotide Domain of Illustrative Sense-Strand Probe for Detecting SARS-CoV-2 ORF1ab
tgcccgtaatggtgttctta

SEQ ID NO: 134 - DNA, 26 bp, SARS-CoV2 Coronavirus
  misc_feature (1)..(26): SARS-CoV-2 Polynucleotide Domain of Illustrative Sense-Strand Probe for Detecting SARS-CoV-2 ORF1ab
gcccgtaatggtgttcttattacaga

SEQ ID NO: 135 - DNA, 25 bp, SARS-CoV2 Coronavirus
  misc_feature (1)..(25): SARS-CoV-2 Polynucleotide Domain of Illustrative Sense-Strand Probe for Detecting SARS-CoV-2 ORF1ab
cccgtaatggtgttcttattacaga

SEQ ID NO: 136 - DNA, 24 bp, SARS-CoV2 Coronavirus
  misc_feature (1)..(24): SARS-CoV-2 Polynucleotide Domain of Illustrative Sense-Strand Probe for Detecting SARS-CoV-2 ORF1ab
ccgtaatggtgttcttattacaga

SEQ ID NO: 137 - DNA, 23 bp, SARS-CoV2 Coronavirus
  misc_feature (1)..(23): SARS-CoV-2 Polynucleotide Domain of Illustrative Sense-Strand Probe for Detecting SARS-CoV-2 ORF1ab
cgtaatggtgttcttattacaga

SEQ ID NO: 138 - DNA, 22 bp, SARS-CoV2 Coronavirus
  misc_feature (1)..(22): SARS-CoV-2 Polynucleotide Domain of Illustrative Sense-Strand Probe for Detecting SARS-CoV-2 ORF1ab
gtaatggtgttcttattacaga

SEQ ID NO: 139 - DNA, 21 bp, SARS-CoV2 Coronavirus
  misc_feature (1)..(21): SARS-CoV-2 Polynucleotide Domain of Illustrative Sense-Strand Probe for Detecting SARS-CoV-2 ORF1ab
taatggtgttcttattacaga

SEQ ID NO: 140 - DNA, 20 bp, SARS-CoV2 Coronavirus
  misc_feature (1)..(20): SARS-CoV-2 Polynucleotide Domain of Illustrative Sense-Strand Probe for Detecting SARS-CoV-2 ORF1ab
aatggtgttcttattacaga

SEQ ID NO: 141 - DNA, 20 bp, SARS-CoV2 Coronavirus
  misc_feature (1)..(20): SARS-CoV-2 Polynucleotide Domain of Illustrative Sense-Strand Probe for Detecting SARS-CoV-2 ORF1ab
ttcttattacagaaggtagt

SEQ ID NO: 142 - DNA, 24 bp, SARS-CoV2 Coronavirus
  misc_feature (1)..(24): SARS-CoV-2 Polynucleotide Domain of Illustrative Sense-Strand Probe for Detecting SARS-CoV-2 ORF1ab
gcccgtaatggtgttcttattaca

SEQ ID NO: 143 - DNA, 23 bp, SARS-CoV2 Coronavirus
  misc_feature (1)..(23): SARS-CoV-2 Polynucleotide Domain of Illustrative Sense-Strand Probe for Detecting SARS-CoV-2 ORF1ab
gcccgtaatggtgttcttattac

SEQ ID NO: 144 - DNA, 22 bp, SARS-CoV2 Coronavirus
  misc_feature (1)..(22): SARS-CoV-2 Polynucleotide Domain of Illustrative Sense-Strand Probe for Detecting SARS-CoV-2 ORF1ab
cccgtaatggtgttcttattac

SEQ ID NO: 145 - DNA, 21 bp, SARS-CoV2 Coronavirus
  misc_feature (1)..(21): SARS-CoV-2 Polynucleotide Domain of Illustrative Sense-Strand Probe for Detecting SARS-CoV-2 ORF1ab
cccgtaatggtgttcttatta

SEQ ID NO: 146 - DNA, 20 bp, SARS-CoV2 Coronavirus
  misc_feature (1)..(20): SARS-CoV-2 Polynucleotide Domain of Illustrative Sense-Strand Probe for Detecting SARS-CoV-2 ORF1ab
ccgtaatggtgttcttatta

SEQ ID NO: 147 - DNA, 26 bp, SARS-CoV2 Coronavirus
  misc_feature (1)..(26): SARS-CoV-2 Polynucleotide Domain of Illustrative Antisense-Strand Probe for Detecting SARS-CoV-2 ORF1ab
tctgtaataagaacaccattacgggc

SEQ ID NO: 148 - DNA, 25 bp, SARS-CoV2 Coronavirus
  misc_feature (1)..(25): SARS-CoV-2 Polynucleotide Domain of Illustrative Antisense-Strand Probe for Detecting SARS-CoV-2 ORF1ab
tctgtaataagaacaccattacggg

SEQ ID NO: 149 - DNA, 24 bp, SARS-CoV2 Coronavirus
  misc_feature (1)..(24): SARS-CoV-2 Polynucleotide Domain of Illustrative Antisense-Strand Probe for Detecting SARS-CoV-2 ORF1ab
tctgtaataagaacaccattacgg

SEQ ID NO: 150 - DNA, 23 bp, SARS-CoV2 Coronavirus
  misc_feature (1)..(23): SARS-CoV-2 Polynucleotide Domain of Illustrative Antisense-Strand Probe for Detecting SARS-CoV-2 ORF1ab
tctgtaataagaacaccattacg

SEQ ID NO: 151 - DNA, 22 bp, SARS-CoV2 Coronavirus
  misc_feature (1)..(22): SARS-CoV-2 Polynucleotide Domain of Illustrative Antisense-Strand Probe for Detecting SARS-CoV-2 ORF1ab
tctgtaataagaacaccattac

SEQ ID NO: 152 - DNA, 21 bp, SARS-CoV2 Coronavirus
  misc_feature (1)..(21): SARS-CoV-2 Polynucleotide Domain of Illustrative Antisense-Strand Probe for Detecting SARS-Cov-2 ORF1ab
tctgtaataagaacaccatta

SEQ ID NO: 153 - DNA, 20 bp, SARS-CoV2 Coronavirus
  misc_feature (1)..(20): SARS-CoV-2 Polynucleotide Domain of Illustrative Antisense-Strand Probe for Detecting SARS-CoV-2 ORF1ab
tctgtaataagaacaccatt

SEQ ID NO: 154 - DNA, 26 bp, SARS-CoV2 Coronavirus
  misc_feature (1)..(26): SARS-CoV-2 Polynucleotide Domain of Illustrative Antisense-Strand Probe for Detecting SARS-CoV-2 ORF1ab
ctgtaataagaacaccattacgggca

SEQ ID NO: 155 - DNA, 25 bp, SARS-CoV2 Coronavirus
  misc_feature (1)..(25): SARS-CoV-2 Polynucleotide Domain of Illustrative Antisense-Strand Probe for Detecting SARS-CoV-2 ORF1ab
tgtaataagaacaccattacgggca

SEQ ID NO: 156 - DNA, 24 bp, SARS-CoV2 Coronavirus
  misc_feature (1)..(24): SARS-CoV-2 Polynucleotide Domain of Illustrative Antisense-Strand Probe for Detecting SARS-CoV-2 ORF1ab
gtaataagaacaccattacgggca

SEQ ID NO: 157 - DNA, 23 bp, SARS-CoV2 Coronavirus
  misc_feature (1)..(23): SARS-CoV-2 Polynucleotide Domain of Illustrative Antisense-Strand Probe for Detecting SARS-CoV-2 ORF1ab
taataagaacaccattacgggca

SEQ ID NO: 158 - DNA, 22 bp, SARS-CoV2 Coronavirus
  misc_feature (1)..(22): SARS-CoV-2 Polynucleotide Domain of Illustrative Antisense-Strand Probe for Detecting SARS-CoV-2 ORF1ab
aataagaacaccattacgggca

SEQ ID NO: 159 - DNA, 21 bp, SARS-CoV2 Coronavirus
  misc_feature (1)..(21): SARS-CoV-2 Polynucleotide Domain of Illustrative Antisense-Strand Probe for Detecting SARS-CoV-2 ORF1ab
ataagaacaccattacgggca

SEQ ID NO: 160 - DNA, 20 bp, SARS-CoV2 Coronavirus
  misc_feature (1)..(20): SARS-CoV-2 Polynucleotide Domain of Illustrative Antisense-Strand Probe for Detecting SARS-CoV-2 ORF1ab
taagaacaccattacgggca

SEQ ID NO: 161 - DNA, 25 bp, SARS-CoV2 Coronavirus
  misc_feature (1)..(25): SARS-CoV-2 Polynucleotide Domain of Illustrative Antisense-Strand Probe for Detecting SARS-CoV-2 ORF1ab
ctgtaataagaacaccattacgggc

SEQ ID NO: 162 - DNA, 24 bp, SARS-CoV2 Coronavirus
  misc_feature (1)..(24): SARS-CoV-2 Polynucleotide Domain of Illustrative Antisense-Strand Probe for Detecting SARS-CoV-2 ORF1ab
tgtaataagaacaccattacgggc

SEQ ID NO: 163 - DNA, 23 bp, SARS-CoV2 Coronavirus
  misc_feature (1)..(23): SARS-CoV-2 Polynucleotide Domain of Illustrative Antisense-Strand Probe for Detecting SARS-CoV-2 ORF1ab
gtaataagaacaccattacgggc

SEQ ID NO: 164 - DNA, 22 bp, SARS-CoV2 Coronavirus
  misc_feature (1)..(22): SARS-CoV-2 Polynucleotide Domain of Illustrative Antisense-Strand Probe for Detecting SARS-CoV-2 ORF1ab
gtaataagaacaccattacggg

SEQ ID NO: 165 - DNA, 21 bp, SARS-CoV2 Coronavirus
  misc_feature (1)..(21): SARS-CoV-2 Polynucleotide Domain of Illustrative Antisense-Strand Probe for Detecting SARS-CoV-2 ORF1ab
taataagaacaccattacggg

SEQ ID NO: 166 - DNA, 20 bp, SARS-CoV2 Coronavirus
  misc_feature (1)..(20): SARS-CoV-2 Polynucleotide Domain of Illustrative Antisense-Strand Probe for Detecting SARS-CoV-2 ORF1ab
taataagaacaccattacgg

SEQ ID NO: 167 - DNA, 31 bp, SARS-CoV2 Coronavirus
  misc_feature (1)..(31): SARS-CoV-2 Polynucleotide Domain of Illustrative Sense-Strand Probe for Detecting the SARS-CoV-2 S Gene
ctgttctttatcaggatgttaactgcacaga

SEQ ID NO: 168 - DNA, 31 bp, SARS-CoV2 Coronavirus
  misc_feature (1)..(31): SARS-CoV-2 Polynucleotide Domain of Illustrative Sense-Strand Probe for Detecting the SARS-CoV-2 S Gene
ctgttctttatcagggtgttaactgcacaga

SEQ ID NO: 169 - DNA, 30 bp, SARS-CoV2 Coronavirus
  misc_feature (1)..(30): SARS-CoV-2 Polynucleotide Domain of Illustrative Sense-Strand Probe for Detecting the SARS-CoV-2 S Gene
tgttctttatcaggatgttaactgcacaga

SEQ ID NO: 170 - DNA, 30 bp, SARS-CoV2 Coronavirus
  misc_feature (1)..(30): SARS-CoV-2 Polynucleotide Domain of Illustrative Sense-Strand Probe for Detecting the SARS-CoV-2 S Gene
tgttctttatcagggtgttaactgcacaga

SEQ ID NO: 171 - DNA, 29 bp, SARS-CoV2 Coronavirus
  misc_feature (1)..(29): SARS-CoV-2 Polynucleotide Domain of Illustrative Sense-Strand Probe for Detecting the SARS-CoV-2 S Gene
gttctttatcaggatgttaactgcacaga

SEQ ID NO: 172 - DNA, 29 bp, SARS-CoV2 Coronavirus
  misc_feature (1)..(29): SARS-CoV-2 Polynucleotide Domain of Illustrative Sense-Strand Probe for Detecting the SARS-CoV-2 S Gene
gttctttatcagggtgttaactgcacaga

SEQ ID NO: 173 - DNA, 28 bp, SARS-CoV2 Coronavirus
  misc_feature (1)..(28): SARS-CoV-2 Polynucleotide Domain of Illustrative Sense-Strand Probe for Detecting the SARS-CoV-2 S Gene
ttctttatcaggatgttaactgcacaga

SEQ ID NO: 174 - DNA, 28 bp, SARS-CoV2 Coronavirus
  misc_feature (1)..(28): SARS-CoV-2 Polynucleotide Domain of Illustrative Sense-Strand Probe for Detecting the SARS-CoV-2 S Gene
ttctttatcagggtgttaactgcacaga

SEQ ID NO: 175 - DNA, 27 bp, SARS-CoV2 Coronavirus
  misc_feature (1)..(27): SARS-CoV-2 Polynucleotide Domain of Illustrative Sense-Strand Probe for Detecting the SARS-CoV-2 S Gene
tctttatcaggatgttaactgcacaga

SEQ ID NO: 176 - DNA, 27 bp, SARS-CoV2 Coronavirus
  misc_feature (1)..(27): SARS-CoV-2 Polynucleotide Domain of Illustrative Sense-Strand Probe for Detecting the SARS-CoV-2 S Gene
tctttatcagggtgttaactgcacaga

SEQ ID NO: 177 - DNA, 26 bp, SARS-CoV2 Coronavirus
  misc_feature (1)..(26): SARS-CoV-2 Polynucleotide Domain of Illustrative Sense-Strand Probe for Detecting the SARS-CoV-2 S Gene
ctttatcaggatgttaactgcacaga

SEQ ID NO: 178 - DNA, 26 bp, SARS-CoV2 Coronavirus
  misc_feature (1)..(26): SARS-CoV-2 Polynucleotide Domain of Illustrative Sense-Strand Probe for Detecting the SARS-CoV-2 S Gene
ctttatcagggtgttaactgcacaga

SEQ ID NO: 179 - DNA, 25 bp, SARS-CoV2 Coronavirus
  misc_feature (1)..(25): SARS-CoV-2 Polynucleotide Domain of Illustrative Sense-Strand Probe for Detecting the SARS-CoV-2 S Gene
tttatcaggatgttaactgcacaga

SEQ ID NO: 180 - DNA, 25 bp, SARS-CoV2 Coronavirus
  misc_feature (1)..(25): SARS-CoV-2 Polynucleotide Domain of Illustrative Sense-Strand Probe for Detecting the SARS-CoV-2 S Gene
tttatcagggtgttaactgcacaga

SEQ ID NO: 181 - DNA, 24 bp, SARS-CoV2 Coronavirus
  misc_feature (1)..(24): SARS-CoV-2 Polynucleotide Domain of Illustrative Sense-Strand Probe for Detecting the SARS-CoV-2 S Gene
ttatcaggatgttaactgcacaga

SEQ ID NO: 182 - DNA, 24 bp, SARS-CoV2 Coronavirus
  misc_feature (1)..(24): SARS-CoV-2 Polynucleotide Domain of Illustrative Sense-Strand Probe for Detecting the SARS-CoV-2 S Gene
ttatcagggtgttaactgcacaga

SEQ ID NO: 183 - DNA, 23 bp, SARS-CoV2 Coronavirus
  misc_feature (1)..(23): SARS-CoV-2 Polynucleotide Domain of Illustrative Sense-Strand Probe for Detecting the SARS-CoV-2 S Gene
tatcaggatgttaactgcacaga

SEQ ID NO: 184 - DNA, 23 bp, SARS-CoV2 Coronavirus
  misc_feature (1)..(23): SARS-CoV-2 Polynucleotide Domain of Illustrative Sense-Strand Probe for Detecting the SARS-CoV-2 S Gene
tatcagggtgttaactgcacaga

SEQ ID NO: 185 - DNA, 22 bp, SARS-CoV2 Coronavirus
  misc_feature (1)..(22): SARS-CoV-2 Polynucleotide Domain of Illustrative Sense-Strand Probe for Detecting the SARS-CoV-2 S Gene
atcaggatgttaactgcacaga

SEQ ID NO: 186 - DNA, 22 bp, SARS-CoV2 Coronavirus
  misc_feature (1)..(22): SARS-CoV-2 Polynucleotide Domain of Illustrative Sense-Strand Probe for Detecting the SARS-CoV-2 S Gene
atcagggtgttaactgcacaga

SEQ ID NO: 187 - DNA, 21 bp, SARS-CoV2 Coronavirus
  misc_feature (1)..(21): SARS-CoV-2 Polynucleotide Domain of Illustrative Sense-Strand Probe for Detecting the SARS-CoV-2 S Gene
tcaggatgttaactgcacaga

SEQ ID NO: 188 - DNA, 21 bp, SARS-CoV2 Coronavirus
  misc_feature (1)..(21): SARS-CoV-2 Polynucleotide Domain of Illustrative Sense-Strand Probe for Detecting the SARS-CoV-2 S Gene
tcagggtgttaactgcacaga

SEQ ID NO: 189 - DNA, 20 bp, SARS-CoV2 Coronavirus
  misc_feature (1)..(20): SARS-CoV-2 Polynucleotide Domain of Illustrative Sense-Strand Probe for Detecting the SARS-CoV-2 S Gene
caggatgttaactgcacaga

SEQ ID NO: 190 - DNA, 20 bp, SARS-CoV2 Coronavirus
  misc_feature (1)..(20): SARS-CoV-2 Polynucleotide Domain of Illustrative Sense-Strand Probe for Detecting the SARS-CoV-2 S Gene
cagggtgttaactgcacaga

SEQ ID NO: 191 - DNA, 30 bp, SARS-CoV2 Coronavirus
  misc_feature (1)..(30): SARS-CoV-2 Polynucleotide Domain of Illustrative Sense-Strand Probe for Detecting the SARS-CoV-2 S Gene
ctgttctttatcaggatgttaactgcacag

SEQ ID NO: 192 - DNA, 30 bp, SARS-CoV2 Coronavirus
  misc_feature (1)..(30): SARS-CoV-2 Polynucleotide Domain of Illustrative Sense-Strand Probe for Detecting the SARS-CoV-2 S Gene
ctgttctttatcagggtgttaactgcacag

SEQ ID NO: 193 - DNA, 29 bp, SARS-CoV2 Coronavirus
  misc_feature (1)..(29): SARS-CoV-2 Polynucleotide Domain of Illustrative Sense-Strand Probe for Detecting the SARS-CoV-2 S Gene
ctgttctttatcaggatgttaactgcaca

SEQ ID NO: 194 - DNA, 29 bp, SARS-CoV2 Coronavirus
  misc_feature (1)..(29): SARS-CoV-2 Polynucleotide Domain of Illustrative Sense-Strand Probe for Detecting the SARS-CoV-2 S Gene
ctgttctttatcagggtgttaactgcaca

SEQ ID NO: 195 - DNA, 28 bp, SARS-CoV2 Coronavirus
  misc_feature (1)..(20): SARS-CoV-2 Polynucleotide Domain of Illustrative Sense-Strand Probe for Detecting the SARS-CoV-2 S Gene
ctgttctttatcaggatgttaactgcac

SEQ ID NO: 196 - DNA, 28 bp, SARS-CoV2 Coronavirus
  misc_feature (1)..(28): SARS-CoV-2 Polynucleotide Domain of Illustrative Sense-Strand Probe for Detecting the SARS-CoV-2 S Gene
ctgttctttatcagggtgttaactgcac

SEQ ID NO: 197 - DNA, 27 bp, SARS-CoV2 Coronavirus
  misc_feature (1)..(27): SARS-CoV-2 Polynucleotide Domain of Illustrative Sense-Strand Probe for Detecting the SARS-CoV-2 S Gene
ctgttctttatcaggatgttaactgca

SEQ ID NO: 198 - DNA, 27 bp, SARS-CoV2 Coronavirus
  misc_feature (1)..(27): SARS-CoV-2 Polynucleotide Domain of Illustrative Sense-Strand Probe for Detecting the SARS-CoV-2 S Gene
ctgttctttatcagggtgttaactgca

SEQ ID NO: 199 - DNA, 26 bp, SARS-CoV2 Coronavirus
  misc_feature (1)..(26): SARS-CoV-2 Polynucleotide Domain of Illustrative Sense-Strand Probe for Detecting the SARS-CoV-2 S Gene
ctgttctttatcaggatgttaactgc

SEQ ID NO: 200 - DNA, 26 bp, SARS-CoV2 Coronavirus
  misc_feature (1)..(26): SARS-CoV-2 Polynucleotide Domain of Illustrative Sense-Strand Probe for Detecting the SARS-CoV-2 S Gene
ctgttctttatcagggtgttaactgc

SEQ ID NO: 201 - DNA, 25 bp, SARS-CoV2 Coronavirus
  misc_feature (1)..(25): SARS-CoV-2 Polynucleotide Domain of Illustrative Sense-Strand Probe for Detecting the SARS-CoV-2 S Gene
ctgttctttatcaggatgttaactg

SEQ ID NO: 202 - DNA, 25 bp, SARS-CoV2 Coronavirus
  misc_feature (1)..(25): SARS-CoV-2 Polynucleotide Domain of Illustrative Sense-Strand Probe for Detecting the SARS-CoV-2 S Gene
ctgttctttatcagggtgttaactg

SEQ ID NO: 203 - DNA, 24 bp, SARS-CoV2 Coronavirus
  misc_feature (1)..(24): SARS-CoV-2 Polynucleotide Domain of Illustrative Sense-Strand Probe for Detecting the SARS-CoV-2 S Gene
ctgttctttatcaggatgttaact

SEQ ID NO: 204 - DNA, 24 bp, SARS-CoV2 Coronavirus
  misc_feature (1)..(24): SARS-CoV-2 Polynucleotide Domain of Illustrative Sense-Strand Probe for Detecting the SARS-CoV-2 S Gene
ctgttctttatcagggtgttaact

SEQ ID NO: 205 - DNA, 23 bp, SARS-CoV2 Coronavirus
  misc_feature (1)..(23): SARS-CoV-2 Polynucleotide Domain of Illustrative Sense-Strand Probe for Detecting the SARS-CoV-2 S Gene
ctgttctttatcaggatgttaac

SEQ ID NO: 206 - DNA, 23 bp, SARS-CoV2 Coronavirus
  misc_feature (1)..(23): SARS-CoV-2 Polynucleotide Domain of Illustrative Sense-Strand Probe for Detecting the SARS-CoV-2 S Gene
ctgttctttatcagggtgttaac

SEQ ID NO: 207 - DNA, 22 bp, SARS-CoV2 Coronavirus
  misc_feature (1)..(22): SARS-CoV-2 Polynucleotide Domain of Illustrative Sense-Strand Probe for Detecting the SARS-CoV-2 S Gene
ctgttctttatcaggatgttaa

SEQ ID NO: 208 - DNA, 22 bp, SARS-CoV2 Coronavirus
  misc_feature (1)..(22): SARS-CoV-2 Polynucleotide Domain of Illustrative Sense-Strand Probe for Detecting the SARS-CoV-2 S Gene
ctgttctttatcagggtgttaa

SEQ ID NO: 209 - DNA, 21 bp, SARS-CoV2 Coronavirus
  misc_feature (1)..(21): SARS-CoV-2 Polynucleotide Domain of Illustrative Sense-Strand Probe for Detecting the SARS-CoV-2 S Gene
ctgttctttatcaggatgtta

SEQ ID NO: 210 - DNA, 21 bp, SARS-CoV2 Coronavirus
  misc_feature (1)..(21): SARS-CoV-2 Polynucleotide Domain of Illustrative Sense-Strand Probe for Detecting the SARS-CoV-2 S Gene
ctgttctttatcagggtgtta

SEQ ID NO: 211 - DNA, 20 bp, SARS-CoV2 Coronavirus
  misc_feature (1)..(20): SARS-CoV-2 Polynucleotide Domain of Illustrative Sense-Strand Probe for Detecting the SARS-CoV-2 S Gene
ctgttctttatcaggatgtt

SEQ ID NO: 212 - DNA, 20 bp, SARS-CoV2 Coronavirus
  misc_feature (1)..(20): SARS-CoV-2 Polynucleotide Domain of Illustrative Sense-Strand Probe for Detecting the SARS-CoV-2 S Gene
ctgttctttatcagggtgtt

SEQ ID NO: 213 - DNA, 30 bp, SARS-CoV2 Coronavirus; identical to SEQ ID NO: 169
  misc_feature (1)..(30): SARS-CoV-2 Polynucleotide Domain of Illustrative Sense-Strand Probe for Detecting the SARS-CoV-2 S Gene

SEQ ID NO: 214 - DNA, 30 bp, SARS-CoV2 Coronavirus; identical to SEQ ID NO: 170
  misc_feature (1)..(30): SARS-CoV-2 Polynucleotide Domain of Illustrative Sense-Strand Probe for Detecting the SARS-CoV-2 S Gene

SEQ ID NO: 215 - DNA, 29 bp, SARS-CoV2 Coronavirus
  misc_feature (1)..(29): SARS-CoV-2 Polynucleotide Domain of Illustrative Sense-Strand Probe for Detecting the SARS-CoV-2 S Gene
tgttctttatcaggatgttaactgcacag

SEQ ID NO: 216 - DNA, 29 bp, SARS-CoV2 Coronavirus
  misc_feature (1)..(29): SARS-CoV-2 Polynucleotide Domain of Illustrative Sense-Strand Probe for Detecting the SARS-CoV-2 S Gene
tgttctttatcagggtgttaactgcacag

SEQ ID NO: 217 - DNA, 28 bp, SARS-CoV2 Coronavirus
  misc_feature (1)..(28): SARS-CoV-2 Polynucleotide Domain of Illustrative Sense-Strand Probe for Detecting the SARS-CoV-2 S Gene
gttctttatcaggatgttaactgcacag

SEQ ID NO: 218 - DNA, 28 bp, SARS-CoV2 Coronavirus
  misc_feature (1)..(28): SARS-CoV-2 Polynucleotide Domain of Illustrative Sense-Strand Probe for Detecting the SARS-CoV-2 S Gene
gttctttatcagggtgttaactgcacag

SEQ ID NO: 219 - DNA, 27 bp, SARS-CoV2 Coronavirus
  misc_feature (1)..(27): SARS-CoV-2 Polynucleotide Domain of Illustrative Sense-Strand Probe for Detecting the SARS-CoV-2 S Gene
gttctttatcaggatgttaactgcaca

SEQ ID NO: 220 - DNA, 27 bp, SARS-CoV2 Coronavirus
  misc_feature (1)..(27): SARS-CoV-2 Polynucleotide Domain of Illustrative Sense-Strand Probe for Detecting the SARS-CoV-2 S Gene
gttctttatcagggtgttaactgcaca

SEQ ID NO: 221 - DNA, 26 bp, SARS-CoV2 Coronavirus
  misc_feature (1)..(26): SARS-CoV-2 Polynucleotide Domain of Illustrative Sense-Strand Probe for Detecting the SARS-CoV-2 S Gene
ttctttatcaggatgttaactgcaca

SEQ ID NO: 222 - DNA, 26 bp, SARS-CoV2 Coronavirus
  misc_feature (1)..(26): SARS-CoV-2 Polynucleotide Domain of Illustrative Sense-Strand Probe for Detecting the SARS-CoV-2 S Gene
ttctttatcagggtgttaactgcaca

SEQ ID NO: 223 - DNA, 25 bp, SARS-CoV2 Coronavirus
  misc_feature (1)..(25): SARS-CoV-2 Polynucleotide Domain of Illustrative Sense-Strand Probe for Detecting the SARS-CoV-2 S Gene
ttctttatcaggatgttaactgcac

SEQ ID NO: 224 - DNA, 25 bp, SARS-CoV2 Coronavirus
  misc_feature (1)..(25): SARS-CoV-2 Polynucleotide Domain of Illustrative Sense-Strand Probe for Detecting the SARS-CoV-2 S Gene
ttctttatcagggtgttaactgcac

SEQ ID NO: 225 - DNA, 24 bp, SARS-CoV2 Coronavirus
  misc_feature (1)..(24): SARS-CoV-2 Polynucleotide Domain of Illustrative Sense-Strand Probe for Detecting the SARS-CoV-2 S Gene
tctttatcaggatgttaactgcac

SEQ ID NO: 226 - DNA, 24 bp, SARS-CoV2 Coronavirus
  misc_feature (1)..(24): SARS-CoV-2 Polynucleotide Domain of Illustrative Sense-Strand Probe for Detecting the SARS-CoV-2 S Gene
tctttatcagggtgttaactgcac

SEQ ID NO: 227 - DNA, 23 bp, SARS-CoV2 Coronavirus
  misc_feature (1)..(23): SARS-CoV-2 Polynucleotide Domain of Illustrative Sense-Strand Probe for Detecting the SARS-CoV-2 S Gene
tctttatcaggatgttaactgca

SEQ ID NO: 228 - DNA, 23 bp, SARS-CoV2 Coronavirus
  misc_feature (1)..(23): SARS-CoV-2 Polynucleotide Domain of Illustrative Sense-Strand Probe for Detecting the SARS-CoV-2 S Gene
tctttatcagggtgttaactgca

SEQ ID NO: 229 - DNA, 22 bp, SARS-CoV2 Coronavirus
  misc_feature (1)..(22): SARS-CoV-2 Polynucleotide Domain of Illustrative Sense-Strand Probe for Detecting the SARS-CoV-2 S Gene
ctttatcaggatgttaactgca

SEQ ID NO: 230 - DNA, 22 bp, SARS-CoV2 Coronavirus
  misc_feature (1)..(22): SARS-CoV-2 Polynucleotide Domain of Illustrative Sense-Strand Probe for Detecting the SARS-CoV-2 S Gene
ctttatcagggtgttaactgca

SEQ ID NO: 231 - DNA, 21 bp, SARS-CoV2 Coronavirus
  misc_feature (1)..(21): SARS-CoV-2 Polynucleotide Domain of Illustrative Sense-Strand Probe for Detecting the SARS-CoV-2 S Gene
ctttatcaggatgttaactgc

SEQ ID NO: 232 - DNA, 21 bp, SARS-CoV2 Coronavirus
  misc_feature (1)..(21): SARS-CoV-2 Polynucleotide Domain of Illustrative Sense-Strand Probe for Detecting the SARS-CoV-2 S Gene
ctttatcagggtgttaactgc

SEQ ID NO: 233 - DNA, 20 bp, SARS-CoV2 Coronavirus
  misc_feature (1)..(20): SARS-CoV-2 Polynucleotide Domain of Illustrative Sense-Strand Probe for Detecting the SARS-CoV-2 S Gene
tttatcaggatgttaactgc

SEQ ID NO: 234 - DNA, 20 bp, SARS-CoV2 Coronavirus
  misc_feature (1)..(20): SARS-CoV-2 Polynucleotide Domain of Illustrative Sense-Strand Probe for Detecting the SARS-CoV-2 S Gene
tttatcagggtgttaactgc

SEQ ID NO: 235 - DNA, 19 bp, SARS-CoV2 Coronavirus
  misc_feature (1)..(19): SARS-CoV-2 Polynucleotide Domain of Illustrative Sense-Strand Probe for Detecting the SARS-CoV-2 S Gene
tttatcaggatgttaactg

SEQ ID NO: 236 - DNA, 19 bp, SARS-CoV2 Coronavirus
  misc_feature (1)..(19): SARS-CoV-2 Polynucleotide Domain of Illustrative Sense-Strand Probe for Detecting the SARS-CoV-2 S Gene
tttatcagggtgttaactg

SEQ ID NO: 237 - DNA, 18 bp, SARS-CoV2 Coronavirus
  misc_feature (1)..(18): SARS-CoV-2 Polynucleotide Domain of Illustrative Sense-Strand Probe for Detecting the SARS-CoV-2 S Gene
ttatcaggatgttaactg

SEQ ID NO: 238 - DNA, 18 bp, SARS-CoV2 Coronavirus
  misc_feature (1)..(18): SARS-CoV-2 Polynucleotide Domain of Illustrative Sense-Strand Probe for Detecting the SARS-CoV-2 S Gene
ttatcagggtgttaactg

SEQ ID NO: 239 - DNA, 17 bp, SARS-CoV2 Coronavirus
  misc_feature (1)..(17): SARS-CoV-2 Polynucleotide Domain of Illustrative Sense-Strand Probe for Detecting the SARS-CoV-2 S Gene
tatcaggatgttaactg

SEQ ID NO: 240 - DNA, 17 bp, SARS-CoV2 Coronavirus
  misc_feature (1)..(17): SARS-CoV-2 Polynucleotide Domain of Illustrative Sense-Strand Probe for Detecting the SARS-CoV-2 S Gene
tatcagggtgttaactg

SEQ ID NO: 241 - DNA, 16 bp, SARS-CoV2 Coronavirus
  misc_feature (1)..(16): SARS-CoV-2 Polynucleotide Domain of Illustrative Sense-Strand Probe for Detecting the SARS-CoV-2 S Gene
tatcaggatgttaact

SEQ ID NO: 242 - DNA, 16 bp, SARS-CoV2 Coronavirus
  misc_feature (1)..(16): SARS-CoV-2 Polynucleotide Domain of Illustrative Sense-Strand Probe for Detecting the SARS-CoV-2 S Gene
tatcagggtgttaact

SEQ ID NO: 243 - DNA, 15 bp, SARS-CoV2 Coronavirus
  misc_feature (1)..(15): SARS-CoV-2 Polynucleotide Domain of Illustrative Sense-Strand Probe for Detecting the SARS-CoV-2 S Gene
atcaggatgttaact

SEQ ID NO: 244 - DNA, 15 bp, SARS-CoV2 Coronavirus
  misc_feature (1)..(15): SARS-CoV-2 Polynucleotide Domain of Illustrative Sense-Strand Probe for Detecting the SARS-CoV-2 S Gene
atcagggtgttaact

SEQ ID NO: 245 - DNA, 14 bp, SARS-CoV2 Coronavirus
  misc_feature (1)..(14): SARS-CoV-2 Polynucleotide Domain of Illustrative Sense-Strand Probe for Detecting the SARS-CoV-2 S Gene
tcaggatgttaact

SEQ ID NO: 246 - DNA, 14 bp, SARS-CoV2 Coronavirus
  misc_feature (1)..(14): SARS-CoV-2 Polynucleotide Domain of Illustrative Sense-Strand Probe for Detecting the SARS-CoV-2 S Gene
tcagggtgttaact

SEQ ID NO: 247 - DNA, 13 bp, SARS-CoV2 Coronavirus
  misc_feature (1)..(13): SARS-CoV-2 Polynucleotide Domain of Illustrative Sense-Strand Probe for Detecting the SARS-CoV-2 S Gene
tcaggatgttaac

SEQ ID NO: 248 - DNA, 13 bp, SARS-CoV2 Coronavirus
  misc_feature (1)..(13): SARS-CoV-2 Polynucleotide Domain of Illustrative Sense-Strand Probe for Detecting the SARS-CoV-2 S Gene
tcagggtgttaac

SEQ ID NO: 249 - DNA, 12 bp, SARS-CoV2 Coronavirus
  misc_feature (1)..(12): SARS-CoV-2 Polynucleotide Domain of Illustrative Sense-Strand Probe for Detecting the SARS-CoV-2 S Gene
tcaggatgttaa

SEQ ID NO: 250 - DNA, 12 bp, SARS-CoV2 Coronavirus
  misc_feature (1)..(12): SARS-CoV-2 Polynucleotide Domain of Illustrative Sense-Strand Probe for Detecting the SARS-CoV-2 S Gene
tcagggtgttaa

SEQ ID NO: 251 - DNA, 11 bp, SARS-CoV2 Coronavirus
  misc_feature (1)..(11): SARS-CoV-2 Polynucleotide Domain of Illustrative Sense-Strand Probe for Detecting the SARS-CoV-2 S Gene
tcaggatgtta

SEQ ID NO: 252 - DNA, 11 bp, SARS-CoV2 Coronavirus
  misc_feature (1)..(11): SARS-CoV-2 Polynucleotide Domain of Illustrative Sense-Strand Probe for Detecting the SARS-CoV-2 S Gene
tcagggtgtta

SEQ ID NO: 253 - DNA, 20 bp, SARS-CoV2 Coronavirus
  misc_feature (1)..(20): SARS-CoV-2 Polynucleotide Domain of Illustrative Sense-Strand Probe for Detecting the SARS-CoV-2 S Gene
gcacagaagtccctgttgct

SEQ ID NO: 254 - DNA, 19 bp, SARS-CoV2 Coronavirus
  misc_feature (1)..(19): SARS-CoV-2 Polynucleotide Domain of Illustrative Sense-Strand Probe for Detecting the SARS-CoV-2 S Gene
cacagaagtccctgttgct

SEQ ID NO: 255 - DNA, 18 bp, SARS-CoV2 Coronavirus
  misc_feature (1)..(18): SARS-CoV-2 Polynucleotide Domain of Illustrative Sense-Strand Probe for Detecting the SARS-CoV-2 S Gene
acagaagtccctgttgct

SEQ ID NO: 256 - DNA, 17 bp, SARS-CoV2 Coronavirus
  misc_feature (1)..(17): SARS-CoV-2 Polynucleotide Domain of Illustrative Sense-Strand Probe for Detecting the SARS-CoV-2 S Gene
cagaagtccctgttgct

SEQ ID NO: 257 - DNA, 20 bp, SARS-CoV2 Coronavirus
  misc_feature (1)..(20): SARS-CoV-2 Polynucleotide Domain of Illustrative Sense-Strand Probe for Detecting the SARS-CoV-2 S Gene
cagaagtccctgttgctatt

SEQ ID NO: 258 - DNA, 16 bp, SARS-CoV2 Coronavirus
  misc_feature (1)..(16): SARS-CoV-2 Polynucleotide Domain of Illustrative Sense-Strand Probe for Detecting the SARS-CoV-2 S Gene
agaagtccctgttgct

SEQ ID NO: 259 - DNA, 15 bp, SARS-CoV2 Coronavirus
  misc_feature (1)..(15): SARS-CoV-2 Polynucleotide Domain of Illustrative Sense-Strand Probe for Detecting the SARS-CoV-2 S Gene
gaagtccctgttgct

SEQ ID NO: 260 - DNA, 20 bp, SARS-CoV2 Coronavirus
  misc_feature (1)..(20): SARS-CoV-2 Polynucleotide Domain of Illustrative Sense-Strand Probe for Detecting the SARS-CoV-2 S Gene
tgcacagaagtccctgttgc

SEQ ID NO: 261 - DNA, 19 bp, SARS-CoV2 Coronavirus
  misc_feature (1)..(19): SARS-CoV-2 Polynucleotide Domain of Illustrative Sense-Strand Probe for Detecting the SARS-CoV-2 S Gene
tgcacagaagtccctgttg

SEQ ID NO: 262 - DNA, 18 bp, SARS-CoV2 Coronavirus
  misc_feature (1)..(18): SARS-CoV-2 Polynucleotide Domain of Illustrative Sense-Strand Probe for Detecting the SARS-CoV-2 S Gene
tgcacagaagtccctgtt

SEQ ID NO: 263 - DNA, 17 bp, SARS-CoV2 Coronavirus
  misc_feature (1)..(17): SARS-CoV-2 Polynucleotide Domain of Illustrative Sense-Strand Probe for Detecting the SARS-CoV-2 S Gene
tgcacagaagtccctgt

SEQ ID NO: 264 - DNA, 16 bp, SARS-CoV2 Coronavirus
  misc_feature (1)..(16): SARS-CoV-2 Polynucleotide Domain of Illustrative Sense-Strand Probe for Detecting the SARS-CoV-2 S Gene
tgcacagaagtccctg

SEQ ID NO: 265 - DNA, 15 bp, SARS-CoV2 Coronavirus
  misc_feature (1)..(15): SARS-CoV-2 Polynucleotide Domain of Illustrative Sense-Strand Probe for Detecting the SARS-CoV-2 S Gene
tgcacagaagtccct

SEQ ID NO: 266 - DNA, 19 bp, SARS-CoV2 Coronavirus
  misc_feature (1)..(19): SARS-CoV-2 Polynucleotide Domain of Illustrative Sense-Strand Probe for Detecting the SARS-CoV-2 S Gene
gcacagaagtccctgttgc

SEQ ID NO: 267 - DNA, 18 bp, SARS-CoV2 Coronavirus
  misc_feature (1)..(18): SARS-CoV-2 Polynucleotide Domain of Illustrative Sense-Strand Probe for Detecting the SARS-CoV-2 S Gene
cacagaagtccctgttgc

SEQ ID NO: 268 - DNA, 17 bp, SARS-CoV2 Coronavirus
  misc_feature (1)..(17): SARS-CoV-2 Polynucleotide Domain of Illustrative Sense-Strand Probe for Detecting the SARS-CoV-2 S Gene
cacagaagtccctgttg

SEQ ID NO: 269 - DNA, 17 bp, SARS-CoV2 Coronavirus
  misc_feature (1)..(17): SARS-CoV-2 Polynucleotide Domain of Illustrative Sense-Strand Probe for Detecting the SARS-CoV-2 S Gene
acagaagtccctgttgc

SEQ ID NO: 270 - DNA, 16 bp, SARS-CoV2 Coronavirus
  misc_feature (1)..(16): SARS-CoV-2 Polynucleotide Domain of Illustrative Sense-Strand Probe for Detecting the SARS-CoV-2 S Gene
acagaagtccctgttg

SEQ ID NO: 271 - DNA, 16 bp, SARS-CoV2 Coronavirus
  misc_feature (1)..(16): SARS-CoV-2 Polynucleotide Domain of Illustrative Sense-Strand Probe for Detecting the SARS-CoV-2 S Gene
cagaagtccctgttgc

SEQ ID NO: 272 - DNA, 15 bp, SARS-CoV2 Coronavirus
  misc_feature (1)..(15): SARS-CoV-2 Polynucleotide Domain of Illustrative Sense-Strand Probe for Detecting the SARS-CoV-2 S Gene
cagaagtccctgttg

SEQ ID NO: 273 - DNA, 31 bp, SARS-CoV2 Coronavirus
  misc_feature (1)..(31): SARS-CoV-2 Polynucleotide Domain of Illustrative Antisense-Strand Probe for Detecting the SARS-CoV-2 S Gene
tctgtgcagttaacatcctgataaagaacag

SEQ ID NO: 274 - DNA, 31 bp, SARS-CoV2 Coronavirus; identical to SEQ ID NO: 273
  misc_feature (1)..(31): SARS-CoV-2 Polynucleotide Domain of Illustrative Antisense-Strand Probe for Detecting the SARS-CoV-2 S Gene

SEQ ID NO: 275 - DNA, 31 bp, SARS-CoV2 Coronavirus
  misc_feature (1)..(31): SARS-CoV-2 Polynucleotide Domain of Illustrative Antisense-Strand Probe for Detecting the SARS-CoV-2 S Gene
tctgtgcagttaacaccctgataaagaacag

SEQ ID NO: 276 - DNA, 30 bp, SARS-CoV2 Coronavirus
  misc_feature (1)..(30): SARS-CoV-2 Polynucleotide Domain of Illustrative Antisense-Strand Probe for Detecting the SARS-CoV-2 S Gene
ctgtgcagttaacatcctgataaagaacag

SEQ ID NO: 277 - DNA, 30 bp, SARS-CoV2 Coronavirus
  misc_feature (1)..(30): SARS-CoV-2 Polynucleotide Domain of Illustrative Antisense-Strand Probe for Detecting the SARS-CoV-2 S Gene
ctgtgcagttaacaccctgataaagaacag

SEQ ID NO: 278 - DNA, 29 bp, SARS-CoV2 Coronavirus
  misc_feature (1)..(29): SARS-CoV-2 Polynucleotide Domain of Illustrative Antisense-Strand Probe for Detecting the SARS-CoV-2 S Gene
tgtgcagttaacatcctgataaagaacag

SEQ ID NO: 279 - DNA, 29 bp, SARS-CoV2 Coronavirus
  misc_feature (1)..(29): SARS-CoV-2 Polynucleotide Domain of Illustrative Antisense-Strand Probe for Detecting the SARS-CoV-2 S Gene
tgtgcagttaacaccctgataaagaacag

SEQ ID NO: 280 - DNA, 28 bp, SARS-CoV2 Coronavirus
  misc_feature (1)..(28): SARS-CoV-2 Polynucleotide Domain of Illustrative Antisense-Strand Probe for Detecting the SARS-CoV-2 S Gene
gtgcagttaacatcctgataaagaacag

SEQ ID NO: 281 - DNA, 28 bp, SARS-CoV2 Coronavirus
  misc_feature (1)..(28): SARS-CoV-2 Polynucleotide Domain of Illustrative Antisense-Strand Probe for Detecting the SARS-CoV-2 S Gene
gtgcagttaacaccctgataaagaacag

SEQ ID NO: 282 - DNA, 27 bp, SARS-CoV2 Coronavirus
  misc_feature (1)..(27): SARS-CoV-2 Polynucleotide Domain of Illustrative Antisense-Strand Probe for Detecting the SARS-CoV-2 S Gene
tgcagttaacatcctgataaagaacag

SEQ ID NO: 283 - DNA, 27 bp, SARS-CoV2 Coronavirus
  misc_feature (1)..(27): SARS-CoV-2 Polynucleotide Domain of Illustrative Antisense-Strand Probe for Detecting the SARS-CoV-2 S Gene
tgcagttaacaccctgataaagaacag

SEQ ID NO: 284 - DNA, 26 bp, SARS-CoV2 Coronavirus
  misc_feature (1)..(26): SARS-CoV-2 Polynucleotide Domain of Illustrative Antisense-Strand Probe for Detecting the SARS-CoV-2 S Gene
gcagttaacatcctgataaagaacag

SEQ ID NO: 285 - DNA, 26 bp, SARS-CoV2 Coronavirus
  misc_feature (1)..(26): SARS-CoV-2 Polynucleotide Domain of Illustrative Antisense-Strand Probe for Detecting the SARS-CoV-2 S Gene
gcagttaacaccctgataaagaacag

SEQ ID NO: 286 - DNA, 25 bp, SARS-CoV2 Coronavirus
  misc_feature (1)..(25): SARS-CoV-2 Polynucleotide Domain of Illustrative Antisense-Strand Probe for Detecting the SARS-CoV-2 S Gene
cagttaacatcctgataaagaacag

SEQ ID NO: 287 - DNA, 25 bp, SARS-CoV2 Coronavirus
  misc_feature (1)..(25): SARS-CoV-2 Polynucleotide Domain of Illustrative Antisense-Strand Probe for Detecting the SARS-CoV-2 S Gene
cagttaacaccctgataaagaacag

SEQ ID NO: 288 - DNA, 24 bp, SARS-CoV2 Coronavirus
  misc_feature (1)..(24): SARS-CoV-2 Polynucleotide Domain of Illustrative Antisense-Strand Probe for Detecting the SARS-CoV-2 S Gene
agttaacatcctgataaagaacag

SEQ ID NO: 289 - DNA, 24 bp, SARS-CoV2 Coronavirus
  misc_feature (1)..(24): SARS-CoV-2 Polynucleotide Domain of Illustrative Antisense-Strand Probe for Detecting the SARS-CoV-2 S Gene
agttaacaccctgataaagaacag

SEQ ID NO: 290 - DNA, 23 bp, SARS-CoV2 Coronavirus
  misc_feature (1)..(23): SARS-CoV-2 Polynucleotide Domain of Illustrative Antisense-Strand Probe for Detecting the SARS-CoV-2 S Gene
gttaacatcctgataaagaacag

SEQ ID NO: 291 - DNA, 23 bp, SARS-CoV2 Coronavirus
  misc_feature (1)..(23): SARS-CoV-2 Polynucleotide Domain of Illustrative Antisense-Strand Probe for Detecting the SARS-CoV-2 S Gene
gttaacaccctgataaagaacag

SEQ ID NO: 292 - DNA, 22 bp, SARS-CoV2 Coronavirus
  misc_feature (1)..(22): SARS-CoV-2 Polynucleotide Domain of Illustrative Antisense-Strand Probe for Detecting the SARS-CoV-2 S Gene
ttaacatcctgataaagaacag

SEQ ID NO: 293 - DNA, 22 bp, SARS-CoV2 Coronavirus
  misc_feature (1)..(22): SARS-CoV-2 Polynucleotide Domain of Illustrative Antisense-Strand Probe for Detecting the SARS-CoV-2 S Gene
ttaacaccctgataaagaacag

SEQ ID NO: 294 - DNA, 21 bp, SARS-CoV2 Coronavirus
  misc_feature (1)..(21): SARS-CoV-2 Polynucleotide Domain of Illustrative Antisense-Strand Probe for Detecting the SARS-CoV-2 S Gene
taacatcctgataaagaacag

SEQ ID NO: 295 - DNA, 21 bp, SARS-CoV2 Coronavirus
  misc_feature (1)..(21): SARS-CoV-2 Polynucleotide Domain of Illustrative Antisense-Strand Probe for Detecting the SARS-CoV-2 S Gene
taacaccctgataaagaacag

SEQ ID NO: 296 - DNA, 20 bp, SARS-CoV2 Coronavirus
  misc_feature (1)..(20): SARS-CoV-2 Polynucleotide Domain of Illustrative Antisense-Strand Probe for Detecting the SARS-CoV-2 S Gene
aacatcctgataaagaacag

SEQ ID NO: 297 - DNA, 20 bp, SARS-CoV2 Coronavirus
  misc_feature (1)..(20): SARS-CoV-2 Polynucleotide Domain of Illustrative Antisense-Strand Probe for Detecting the SARS-CoV-2 S Gene
aacaccctgataaagaacag

SEQ ID NO: 298 - DNA, 30 bp, SARS-CoV2 Coronavirus
  misc_feature (1)..(30): SARS-CoV-2 Polynucleotide Domain of Illustrative Antisense-Strand Probe for Detecting the SARS-CoV-2 S Gene
tctgtgcagttaacatcctgataaagaaca

SEQ ID NO: 299 - DNA, 30 bp, SARS-CoV2 Coronavirus
  misc_feature (1)..(30): SARS-CoV-2 Polynucleotide Domain of Illustrative Antisense-Strand Probe for Detecting the SARS-CoV-2 S Gene
tctgtgcagttaacaccctgataaagaaca

SEQ ID NO: 300 - DNA, 29 bp, SARS-CoV2 Coronavirus
  misc_feature (1)..(29): SARS-CoV-2 Polynucleotide Domain of Illustrative Antisense-Strand Probe for Detecting the SARS-CoV-2 S Gene
tctgtgcagttaacatcctgataaagaac

SEQ ID NO: 301 - DNA, 29 bp, SARS-CoV2 Coronavirus
  misc_feature (1)..(29): SARS-CoV-2 Polynucleotide Domain of Illustrative Antisense-Strand Probe for Detecting the SARS-CoV-2 S Gene
tctgtgcagttaacaccctgataaagaac

SEQ ID NO: 302 - DNA, 28 bp, SARS-CoV2 Coronavirus
  misc_feature (1)..(28): SARS-CoV-2 Polynucleotide Domain of Illustrative Antisense-Strand Probe for Detecting the SARS-CoV-2 S Gene
tctgtgcagttaacatcctgataaagaa

SEQ ID NO: 303 - DNA, 28 bp, SARS-CoV2 Coronavirus
  misc_feature (1)..(28): SARS-CoV-2 Polynucleotide Domain of Illustrative Antisense-Strand Probe for Detecting the SARS-CoV-2 S Gene
tctgtgcagttaacaccctgataaagaa

SEQ ID NO: 304 - DNA, 27 bp, SARS-CoV2 Coronavirus
  misc_feature (1)..(27): SARS-CoV-2 Polynucleotide Domain of Illustrative Antisense-Strand Probe for Detecting the SARS-CoV-2 S Gene
tctgtgcagttaacatcctgataaaga

SEQ ID NO: 305 - DNA, 27 bp, SARS-CoV2 Coronavirus
  misc_feature (1)..(27): SARS-CoV-2 Polynucleotide Domain of Illustrative Antisense-Strand Probe for Detecting the SARS-CoV-2 S Gene
tctgtgcagttaacaccctgataaaga

SEQ ID NO: 306 - DNA, 26 bp, SARS-CoV2 Coronavirus
  misc_feature (1)..(26): SARS-CoV-2 Polynucleotide Domain of Illustrative Antisense-Strand Probe for Detecting the SARS-CoV-2 S Gene
tctgtgcagttaacatcctgataaag

SEQ ID NO: 307 - DNA, 26 bp, SARS-CoV2 Coronavirus
  misc_feature (1)..(26): SARS-CoV-2 Polynucleotide Domain of Illustrative Antisense-Strand Probe for Detecting the SARS-CoV-2 S Gene
tctgtgcagttaacaccctgataaag

SEQ ID NO: 308 - DNA, 25 bp, SARS-CoV2 Coronavirus
  misc_feature (1)..(25): SARS-CoV-2 Polynucleotide Domain of Illustrative Antisense-Strand Probe for Detecting the SARS-CoV-2 S Gene
tctgtgcagttaacatcctgataaa

SEQ ID NO: 309 - DNA, 25 bp, SARS-CoV2 Coronavirus
  misc_feature (1)..(25): SARS-CoV-2 Polynucleotide Domain of Illustrative Antisense-Strand Probe for Detecting the SARS-CoV-2 S Gene
tctgtgcagttaacaccctgataaa

SEQ ID NO: 310 - DNA, 24 bp, SARS-CoV2 Coronavirus
  misc_feature (1)..(24): SARS-CoV-2 Polynucleotide Domain of Illustrative Antisense-Strand Probe for Detecting the SARS-CoV-2 S Gene
tctgtgcagttaacatcctgataa

SEQ ID NO: 311 - DNA, 24 bp, SARS-CoV2 Coronavirus
  misc_feature (1)..(24): SARS-CoV-2 Polynucleotide Domain of Illustrative Antisense-Strand Probe for Detecting the SARS-CoV-2 S Gene
tctgtgcagttaacaccctgataa

SEQ ID NO: 312 - DNA, 23 bp, SARS-CoV2 Coronavirus
  misc_feature (1)..(23): SARS-CoV-2 Polynucleotide Domain of Illustrative Antisense-Strand Probe for Detecting the SARS-CoV-2 S Gene
tctgtgcagttaacatcctgata

SEQ ID NO: 313 - DNA, 23 bp, SARS-CoV2 Coronavirus
  misc_feature (1)..(23): SARS-CoV-2 Polynucleotide Domain of Illustrative Antisense-Strand Probe for Detecting the SARS-CoV-2 S Gene
tctgtgcagttaacaccctgata

SEQ ID NO: 314 - DNA, 22 bp, SARS-CoV2 Coronavirus
  misc_feature (1)..(22): SARS-CoV-2 Polynucleotide Domain of Illustrative Antisense-Strand Probe for Detecting the SARS-CoV-2 S Gene
tctgtgcagttaacatcctgat

SEQ ID NO: 315 - DNA, 22 bp, SARS-CoV2 Coronavirus
  misc_feature (1)..(22): SARS-CoV-2 Polynucleotide Domain of Illustrative Antisense-Strand Probe for Detecting the SARS-CoV-2 S Gene
tctgtgcagttaacaccctgat

SEQ ID NO: 316 - DNA, 21 bp, SARS-CoV2 Coronavirus
  misc_feature (1)..(21): SARS-CoV-2 Polynucleotide Domain of Illustrative Antisense-Strand Probe for Detecting the SARS-CoV-2 S Gene
tctgtgcagttaacatcctga

SEQ ID NO: 317 - DNA, 21 bp, SARS-CoV2 Coronavirus
  misc_feature (1)..(21): SARS-CoV-2 Polynucleotide Domain of Illustrative Antisense-Strand Probe for Detecting the SARS-CoV-2 S Gene
tctgtgcagttaacaccctga

SEQ ID NO: 318 - DNA, 20 bp, SARS-CoV2 Coronavirus
  misc_feature (1)..(20): SARS-CoV-2 Polynucleotide Domain of Illustrative Antisense-Strand Probe for Detecting the SARS-CoV-2 S Gene
tctgtgcagttaacatcctg

SEQ ID NO: 319 - DNA, 20 bp, SARS-CoV2 Coronavirus
  misc_feature (1)..(20): SARS-CoV-2 Polynucleotide Domain of Illustrative Antisense-Strand Probe for Detecting the SARS-CoV-2 S Gene
tctgtgcagttaacaccctg

SEQ ID NO: 320 - DNA, 30 bp, SARS-CoV2 Coronavirus; identical to SEQ ID NO: 276
  misc_feature (1)..(30): SARS-CoV-2 Polynucleotide Domain of Illustrative Antisense-Strand Probe for Detecting the SARS-CoV-2 S Gene

SEQ ID NO: 321 - DNA, 30 bp, SARS-CoV2 Coronavirus; identical to SEQ ID NO: 277
  misc_feature (1)..(30): SARS-CoV-2 Polynucleotide Domain of Illustrative Antisense-Strand Probe for Detecting the SARS-CoV-2 S Gene

SEQ ID NO: 322 - DNA, 29 bp, SARS-CoV2 Coronavirus
  misc_feature (1)..(29): SARS-CoV-2 Polynucleotide Domain of Illustrative Antisense-Strand Probe for Detecting the SARS-CoV-2 S Gene
ctgtgcagttaacatcctgataaagaaca

SEQ ID NO: 323 - DNA, 29 bp, SARS-CoV2 Coronavirus
  misc_feature (1)..(29): SARS-CoV-2 Polynucleotide Domain of Illustrative Antisense-Strand Probe for Detecting the SARS-CoV-2 S Gene
ctgtgcagttaacaccctgataaagaaca

SEQ ID NO: 324 - DNA, 28 bp, SARS-CoV2 Coronavirus
  misc_feature (1)..(28): SARS-CoV-2 Polynucleotide Domain of Illustrative Antisense-Strand Probe for Detecting the SARS-CoV-2 S Gene
tgtgcagttaacatcctgataaagaaca

SEQ ID NO: 325 - DNA, 28 bp, SARS-CoV2 Coronavirus
  misc_feature (1)..(28): SARS-CoV-2 Polynucleotide Domain of Illustrative Antisense-Strand Probe for Detecting the SARS-CoV-2 S Gene
tgtgcagttaacaccctgataaagaaca

SEQ ID NO: 326 - DNA, 27 bp, SARS-CoV2 Coronavirus
  misc_feature (1)..(27): SARS-CoV-2 Polynucleotide Domain of Illustrative Antisense-Strand Probe for Detecting the SARS-CoV-2 S Gene
tgtgcagttaacatcctgataaagaac

SEQ ID NO: 327 - DNA, 27 bp, SARS-CoV2 Coronavirus
  misc_feature (1)..(27): SARS-CoV-2 Polynucleotide Domain of Illustrative Antisense-Strand Probe for Detecting the SARS-CoV-2 S Gene
tgtgcagttaacaccctgataaagaac

SEQ ID NO: 328 - DNA, 26 bp, SARS-CoV2 Coronavirus
  misc_feature (1)..(26): SARS-CoV-2 Polynucleotide Domain of Illustrative Antisense-Strand Probe for Detecting the SARS-CoV-2 S Gene
gtgcagttaacatcctgataaagaac

SEQ ID NO: 329 - DNA, 26 bp, SARS-CoV2 Coronavirus
  misc_feature (1)..(26): SARS-CoV-2 Polynucleotide Domain of Illustrative Antisense-Strand Probe for Detecting the SARS-CoV-2 S Gene
gtgcagttaacaccctgataaagaac

SEQ ID NO: 330 - DNA, 25 bp, SARS-CoV2 Coronavirus
  misc_feature (1)..(25): SARS-CoV-2 Polynucleotide Domain of Illustrative Antisense-Strand Probe for Detecting the SARS-CoV-2 S Gene
gtgcagttaacatcctgataaagaa

SEQ ID NO: 331 - DNA, 25 bp, SARS-CoV2 Coronavirus
  misc_feature (1)..(25): SARS-CoV-2 Polynucleotide Domain of Illustrative Antisense-Strand Probe for Detecting the SARS-CoV-2 S Gene
gtgcagttaacaccctgataaagaa

SEQ ID NO: 332 - DNA, 24 bp, SARS-CoV2 Coronavirus
  misc_feature (1)..(24): SARS-CoV-2 Polynucleotide Domain of Illustrative Antisense-Strand Probe for Detecting the SARS-CoV-2 S Gene
tgcagttaacatcctgataaagaa

SEQ ID NO: 333 - DNA, 24 bp, SARS-CoV2 Coronavirus
  misc_feature (1)..(24): SARS-CoV-2 Polynucleotide Domain of Illustrative Antisense-Strand Probe for Detecting the SARS-CoV-2 S Gene
tgcagttaacaccctgataaagaa

SEQ ID NO: 334 - DNA, 23 bp, SARS-CoV2 Coronavirus
  misc_feature (1)..(23): SARS-CoV-2 Polynucleotide Domain of Illustrative Antisense-Strand Probe for Detecting the SARS-CoV-2 S Gene
tgcagttaacatcctgataaaga

SEQ ID NO: 335 - DNA, 23 bp, SARS-CoV2 Coronavirus
  misc_feature (1)..(23): SARS-CoV-2 Polynucleotide Domain of Illustrative Antisense-Strand Probe for Detecting the SARS-CoV-2 S Gene
tgcagttaacaccctgataaaga

SEQ ID NO: 336 - DNA, 22 bp, SARS-CoV2 Coronavirus
  misc_feature (1)..(22): SARS-CoV-2 Polynucleotide Domain of Illustrative Antisense-Strand Probe for Detecting the SARS-CoV-2 S Gene
gcagttaacatcctgataaaga

SEQ ID NO: 337 - DNA, 22 bp, SARS-CoV2 Coronavirus
  misc_feature (1)..(22): SARS-CoV-2 Polynucleotide Domain of Illustrative Antisense-Strand Probe for Detecting the SARS-CoV-2 S Gene
gcagttaacaccctgataaaga

SEQ ID NO: 338 - DNA, 21 bp, SARS-CoV2 Coronavirus
  misc_feature (1)..(21): SARS-CoV-2 Polynucleotide Domain of Illustrative Antisense-Strand Probe for Detecting the SARS-CoV-2 S Gene
cagttaacatcctgataaaga

SEQ ID NO: 339 - DNA, 21 bp, SARS-CoV2 Coronavirus
  misc_feature (1)..(21): SARS-CoV-2 Polynucleotide Domain of Illustrative Antisense-Strand Probe for Detecting the SARS-CoV-2 S Gene
cagttaacaccctgataaaga

SEQ ID NO: 340 - DNA, 20 bp, SARS-CoV2 Coronavirus
  misc_feature (1)..(20): SARS-CoV-2 Polynucleotide Domain of Illustrative Antisense-Strand Probe for Detecting the SARS-CoV-2 S Gene
agttaacatcctgataaaga

SEQ ID NO: 341 - DNA, 20 bp, SARS-CoV2 Coronavirus
  misc_feature (1)..(20): SARS-CoV-2 Polynucleotide Domain of Illustrative Antisense-Strand Probe for Detecting the SARS-CoV-2 S Gene
agttaacaccctgataaaga

SEQ ID NO: 342 - DNA, 19 bp, SARS-CoV2 Coronavirus
  misc_feature (1)..(19): SARS-CoV-2 Polynucleotide Domain of Illustrative Antisense-Strand Probe for Detecting the SARS-CoV-2 S Gene
agttaacatcctgataaag

SEQ ID NO: 343 - DNA, 19 bp, SARS-CoV2 Coronavirus
  misc_feature (1)..(19): SARS-CoV-2 Polynucleotide Domain of Illustrative Antisense-Strand Probe for Detecting the SARS-CoV-2 S Gene
agttaacaccctgataaag

SEQ ID NO: 344 - DNA, 18 bp, SARS-CoV2 Coronavirus
  misc_feature (1)..(18): SARS-CoV-2 Polynucleotide Domain of Illustrative Antisense-Strand Probe for Detecting the SARS-CoV-2 S Gene
gttaacatcctgataaag

SEQ ID NO: 345 - DNA, 18 bp, SARS-CoV2 Coronavirus
  misc_feature (1)..(18): SARS-CoV-2 Polynucleotide Domain of Illustrative Antisense-Strand Probe for Detecting the SARS-CoV-2 S Gene
gttaacaccctgataaag

SEQ ID NO: 346 - DNA, 17 bp, SARS-CoV2 Coronavirus
  misc_feature (1)..(17): SARS-CoV-2 Polynucleotide Domain of Illustrative Antisense-Strand Probe for Detecting the SARS-CoV-2 S Gene
gttaacatcctgataaa

SEQ ID NO: 347 - DNA, 17 bp, SARS-CoV2 Coronavirus
  misc_feature (1)..(17): SARS-CoV-2 Polynucleotide Domain of Illustrative Antisense-Strand Probe for Detecting the SARS-CoV-2 S Gene
gttaacaccctgataaa

SEQ ID NO: 348 - DNA, 16 bp, SARS-CoV2 Coronavirus
  misc_feature (1)..(16): SARS-CoV-2 Polynucleotide Domain of Illustrative Antisense-Strand Probe for Detecting the SARS-CoV-2 S Gene
ttaacatcctgataaa

SEQ ID NO: 349 - DNA, 16 bp, SARS-CoV2 Coronavirus
  misc_feature (1)..(16): SARS-CoV-2 Polynucleotide Domain of Illustrative Antisense-Strand Probe for Detecting the SARS-CoV-2 S Gene
ttaacaccctgataaa

SEQ ID NO: 350 - DNA, 15 bp, SARS-CoV2 Coronavirus
  misc_feature (1)..(15): SARS-CoV-2 Polynucleotide Domain of Illustrative Antisense-Strand Probe for Detecting the SARS-CoV-2 S Gene
ttaacatcctgataa

SEQ ID NO: 351 - DNA, 15 bp, SARS-CoV2 Coronavirus
  misc_feature (1)..(15): SARS-CoV-2 Polynucleotide Domain of Illustrative Antisense-Strand Probe for Detecting the SARS-CoV-2 S Gene
ttaacaccctgataa

SEQ ID NO: 352 - DNA, 14 bp, SARS-CoV2 Coronavirus
  misc_feature (1)..(14): SARS-CoV-2 Polynucleotide Domain of Illustrative Antisense-Strand Probe for Detecting the SARS-CoV-2 S Gene
taacatcctgataa

SEQ ID NO: 353 - DNA, 14 bp, SARS-CoV2 Coronavirus
  misc_feature (1)..(14): SARS-CoV-2 Polynucleotide Domain of Illustrative Antisense-Strand Probe for Detecting the SARS-CoV-2 S Gene
taacaccctgataa

SEQ ID NO: 354 - DNA, 13 bp, SARS-CoV2 Coronavirus
  misc_feature (1)..(13): SARS-CoV-2 Polynucleotide Domain of Illustrative Antisense-Strand Probe for Detecting the SARS-CoV-2 S Gene
taacatcctgata

SEQ ID NO: 355 - DNA, 13 bp, SARS-CoV2 Coronavirus
  misc_feature (1)..(13): SARS-CoV-2 Polynucleotide Domain of Illustrative Antisense-Strand Probe for Detecting the SARS-CoV-2 S Gene
taacaccctgata

SEQ ID NO: 356 - DNA, 12 bp, SARS-CoV2 Coronavirus
  misc_feature (1)..(12): SARS-CoV-2 Polynucleotide Domain of Illustrative Antisense-Strand Probe for Detecting the SARS-CoV-2 S Gene
taacatcctgat

SEQ ID NO: 357 - DNA, 12 bp, SARS-CoV2 Coronavirus
  misc_feature (1)..(12): SARS-CoV-2 Polynucleotide Domain of Illustrative Antisense-Strand Probe for Detecting the SARS-CoV-2 S Gene
taacaccctgat

SEQ ID NO: 358 - DNA, 10 bp, SARS-CoV2 Coronavirus
  misc_feature (1)..(10): SARS-CoV-2 Polynucleotide Domain of Illustrative Antisense-Strand Probe for Detecting the SARS-CoV-2 S Gene
taacatcctg

SEQ ID NO: 359 - DNA, 10 bp, SARS-CoV2 Coronavirus
  misc_feature (1)..(10): SARS-CoV-2 Polynucleotide Domain of Illustrative Antisense-Strand Probe for Detecting the SARS-CoV-2 S Gene
taacaccctg

SEQ ID NO: 360 - DNA, 11 bp, SARS-CoV2 Coronavirus
  misc_feature (1)..(11): SARS-CoV-2 Polynucleotide Domain of Illustrative Antisense-Strand Probe for Detecting the SARS-CoV-2 S Gene
aacatcctgat

SEQ ID NO: 361 - DNA, 11 bp, SARS-CoV2 Coronavirus
  misc_feature (1)..(11): SARS-CoV-2 Polynucleotide Domain of Illustrative Antisense-Strand Probe for Detecting the SARS-CoV-2 S Gene
aacaccctgat

SEQ ID NO: 362 - DNA, 10 bp, SARS-CoV2 Coronavirus
  misc_feature (1)..(10): SARS-CoV-2 Polynucleotide Domain of Illustrative Antisense-Strand Probe for Detecting the SARS-CoV-2 S Gene
aacatcctga

SEQ ID NO: 363 - DNA, 10 bp, SARS-CoV2 Coronavirus
  misc_feature (1)..(10): SARS-CoV-2 Polynucleotide Domain of Illustrative Antisense-Strand Probe for Detecting the SARS-CoV-2 S Gene
aacaccctga

SEQ ID NO: 364 - DNA, 20 bp, SARS-CoV2 Coronavirus
  misc_feature (1)..(20): SARS-CoV-2 Polynucleotide Domain of Illustrative Antisense-Strand Probe for Detecting the SARS-CoV-2 S Gene
gcaacagggacttctgtgca

SEQ ID NO: 365 - DNA, 19 bp, SARS-CoV2 Coronavirus
  misc_feature (1)..(19): SARS-CoV-2 Polynucleotide Domain of Illustrative Antisense-Strand Probe for Detecting the SARS-CoV-2 S Gene
caacagggacttctgtgca

SEQ ID NO: 366 - DNA, 18 bp, SARS-CoV2 Coronavirus
  misc_feature (1)..(18): SARS-CoV-2 Polynucleotide Domain of Illustrative Antisense-Strand Probe for Detecting the SARS-CoV-2 S Gene
aacagggacttctgtgca

SEQ ID NO: 367 - DNA, 17 bp, SARS-CoV2 Coronavirus
  misc_feature (1)..(17): SARS-CoV-2 Polynucleotide Domain of Illustrative Antisense-Strand Probe for Detecting the SARS-CoV-2 S Gene
acagggacttctgtgca

SEQ ID NO: 368 - DNA, 16 bp, SARS-CoV2 Coronavirus
  misc_feature (1)..(16): SARS-CoV-2 Polynucleotide Domain of Illustrative Antisense-Strand Probe for Detecting the SARS-CoV-2 S Gene
cagggacttctgtgca

SEQ ID NO: 369 - DNA, 15 bp, SARS-CoV2 Coronavirus
  misc_feature (1)..(15): SARS-CoV-2 Polynucleotide Domain of Illustrative Antisense-Strand Probe for Detecting the SARS-CoV-2 S Gene
agggacttctgtgca

SEQ ID NO: 370 - DNA, 20 bp, SARS-CoV2 Coronavirus
  misc_feature (1)..(20): SARS-CoV-2 Polynucleotide Domain of Illustrative Antisense-Strand Probe for Detecting the SARS-CoV-2 S Gene
agcaacagggacttctgtgc

SEQ ID NO: 371 - DNA, 19 bp, SARS-CoV2 Coronavirus
  misc_feature (1)..(19): SARS-CoV-2 Polynucleotide Domain of Illustrative Antisense-Strand Probe for Detecting the SARS-CoV-2 S Gene
agcaacagggacttctgtg

SEQ ID NO: 372 - DNA, 18 bp, SARS-CoV2 Coronavirus
  misc_feature (1)..(18): SARS-CoV-2 Polynucleotide Domain of Illustrative Antisense-Strand Probe for Detecting the SARS-CoV-2 S Gene
agcaacagggacttctgt

SEQ ID NO: 373 - DNA, 17 bp, SARS-CoV2 Coronavirus
  misc_feature (1)..(17): SARS-CoV-2 Polynucleotide Domain of Illustrative Antisense-Strand Probe for Detecting the SARS-CoV-2 S Gene
agcaacagggacttctg

SEQ ID NO: 374 - DNA, 16 bp, SARS-CoV2 Coronavirus
  misc_feature (1)..(16): SARS-CoV-2 Polynucleotide Domain of Illustrative Antisense-Strand Probe for Detecting the SARS-CoV-2 S Gene
agcaacagggacttct

SEQ ID NO: 375 - DNA, 15 bp, SARS-CoV2 Coronavirus
  misc_feature (1)..(15): SARS-CoV-2 Polynucleotide Domain of Illustrative Antisense-Strand Probe for Detecting the SARS-CoV-2 S Gene
agcaacagggacttc

SEQ ID NO: 376 - DNA, 20 bp, SARS-CoV2 Coronavirus
  misc_feature (1)..(20): SARS-CoV-2 Polynucleotide Domain of Illustrative Antisense-Strand Probe for Detecting the SARS-CoV-2 S Gene
gcaacagggacttctgtgca

SEQ ID NO: 377 - DNA, 19 bp, SARS-CoV2 Coronavirus
  misc_feature (1)..(19): SARS-CoV-2 Polynucleotide Domain of Illustrative Antisense-Strand Probe for Detecting the SARS-CoV-2 S Gene
gcaacagggacttctgtgc

SEQ ID NO: 378 - DNA, 18 bp, SARS-CoV2 Coronavirus
  misc_feature (1)..(18): SARS-CoV-2 Polynucleotide Domain of Illustrative Antisense-Strand Probe for Detecting the SARS-CoV-2 S Gene
caacagggacttctgtgc

SEQ ID NO: 379 - DNA, 17 bp, SARS-CoV2 Coronavirus
  misc_feature (1)..(17): SARS-CoV-2 Polynucleotide Domain of Illustrative Antisense-Strand Probe for Detecting the SARS-CoV-2 S Gene
caacagggacttctgtg

SEQ ID NO: 380 - DNA, 16 bp, SARS-CoV2 Coronavirus
  misc_feature (1)..(16): SARS-CoV-2 Polynucleotide Domain of Illustrative Antisense-Strand Probe for Detecting the SARS-CoV-2 S Gene
aacagggacttctgtg

SEQ ID NO: 381 - DNA, 15 bp, SARS-CoV2 Coronavirus
  misc_feature (1)..(15): SARS-CoV-2 Polynucleotide Domain of Illustrative Antisense-Strand Probe for Detecting the SARS-CoV-2 S Gene
aacagggacttctgt

SEQ ID NO: 382-397 - skipped (16 entries)

SEQ ID NO: 398 - DNA, 20 bp, SARS-CoV2 Coronavirus
  misc_feature (1)..(20): PCR Primer Oligonucleotide of Illustrative SARS-CoV-2 ORF1ab Scorpion Primer-Probe
gagttgatggtcaagtagac

SEQ ID NO: 399 - DNA, 20 bp, SARS-CoV2 Coronavirus
  misc_feature (1)..(20): PCR Primer Oligonucleotide of Illustrative SARS-CoV-2 ORF1ab Scorpion Primer-Probe
gtagacttatttagaaatgc

SEQ ID NO: 400 - DNA, 20 bp, SARS-CoV2 Coronavirus
  misc_feature (1)..(20): PCR Primer Oligonucleotide of Illustrative SARS-CoV-2 S Gene Scorpion Primer-Probe
ccaggttgctgttctttatc

SEQ ID NO: 401 - DNA, 20 bp, SARS-CoV2 Coronavirus
  misc_feature (1)..(20): PCR Primer Oligonucleotide of Illustrative SARS-CoV-2 S Gene Scorpion Primer-Probe
gttgctgttctttatcagga

SEQ ID NO: 402 - DNA, 20 bp, SARS-CoV2 Coronavirus
  misc_feature (1)..(20): PCR Primer Oligonucleotide of Illustrative SARS-CoV-2 S Gene Scorpion Primer-Probe
gttgctgttctttatcaggg

SEQ ID NO: 403 - DNA, 45 bp, SARS-CoV2 Coronavirus
  misc_feature (1)..(45): Illustrative LAMP ORF1ab FIP Primer
gaacaccattacgggcatttctatcttttttgatggtagagttga

SEQ ID NO: 404 - DNA, 18 bp, SARS-CoV2 Coronavirus
  misc_feature (1)..(18): Illustrative LAMP ORF1ab F3 Primer
tttgtgcaccactcactg

SEQ ID NO: 405 - DNA, 50 bp, SARS-CoV2 Coronavirus
  misc_feature (1)..(50): Illustrative LAMP ORF1ab BIP Primer
aggtagtgttaaaggtttacaaccacaattaatgtgactccattaagact

SEQ ID NO: 406 - DNA, 20 bp, SARS-CoV2 Coronavirus
  misc_feature (1)..(20): Illustrative LAMP ORF1ab B3 Primer
ctgtgtttttacggcttctc

SEQ ID NO: 407 - DNA, 47 bp, SARS-CoV2 Coronavirus
  misc_feature (1)..(47): Illustrative LAMP S Gene FIP Primer
ctgtgcagttaacatcctgataaagagtgttataacaccaggaacaa

SEQ ID NO: 408 - DNA, 19 bp, SARS-CoV2 Coronavirus
  misc_feature (1)..(19): Illustrative LAMP S Gene F3 Primer
tgttcttttggtggtgtca

SEQ ID NO: 409 - DNA, 46 bp, SARS-CoV2 Coronavirus
  misc_feature (1)..(46): Illustrative LAMP S Gene BIP Primer
gaagtccctgttgctattcatgcgtgtttgaaaaacattagaacct

SEQ ID NO: 410 - DNA, 18 bp, SARS-CoV2 Coronavirus
  misc_feature (1)..(18): Illustrative LAMP S Gene B3 Primer
gcccctattaaacagcct

SEQ ID NO: 411 - DNA, 144 bp, SARS-CoV2 Coronavirus
  misc_feature (1)..(144): SARS-CoV-2 ORF1ab Domain Amplified by Illustrative ORF1ab LAMP Primers
tcttttttgatggtagagttgatggtcaagtagacttatttagaaatgcccgtaatggtgttcttattacagaaggtagtgttaaaggtttacaaccatctgtaggtcccaaacaagctagtcttaatggagtcacattaattg

SEQ ID NO: 412 - DNA, 144 bp, SARS-CoV2 Coronavirus
  misc_feature (1)..(154): Complement SARS-CoV-2 ORF1ab Domain Amplified by Illustrative ORF1ab LAMP Primers
caattaatgtgactccattaagactagcttgtttgggacctacagatggttgtaaacctttaacactaccttctgtaataagaacaccattacgggcatttctaaataagtctacttgaccatcaactctaccatcaaaaaaga

SEQ ID NO: 413 - DNA, 154 bp, SARS-CoV2 Coronavirus
  misc_feature (1)..(154): SARS-CoV-2 S Gene Domain Amplified by Illustrative S Gene LAMP Primers
gtgttataacaccaggaacaaatacttctaaccaggttgctgttctttatcaggatgttaactgcacagaagtccctgttgctattcatgcagatcaacttactcctacttggcgtgtttattctacaggttctaatgtttttcaaacacgtgc

SEQ ID NO: 414 - DNA, 154 bp, SARS-CoV2 Coronavirus
  misc_feature (1)..(154): Complement SARS-CoV-2 S Gene Domain Amplified by Illustrative S Gene LAMP Primers
gcacgtgtttgaaaaacattagaacctgtagaataaacacgccaagtaggagtaagttgatctgcatgaatagcaacagggacttctgtgcagttaacatcctgataaagaacagcaacctggttagaagtatttgttcctggtgttataacac

SEQ ID NO: 415 - DNA, 21290 bp, SARS-CoV2 Coronavirus
  misc_feature (1)..(21290): ORF1ab of SARS-CoV-2 of of GenBank NC_045512
atggagagccttgtccctggtttcaacgagaaaacacacgtccaactcagtttgcctgttttacaggttcgcgacgtgctcgtacgtggctttggagactccgtggaggaggtcttatcagaggcacgtcaacatcttaaagatggcacttgtggcttagtagaagttgaaaaaggcgttttgcctcaacttgaacagccctatgtgttcatcaaacgttcggatgctcgaactgcacctcatggtcatgttatggttgagctggtagcagaactcgaaggcattcagtacggtcgtagtggtgagacacttggtgtccttgtccctcatgtgggcgaaataccagtggcttaccgcaaggttcttcttcgtaagaacggtaataaaggagctggtggccatagttacggcgccgatctaaagtcatttgacttaggcgacgagcttggcactgatccttatgaagattttcaagaaaactggaacactaaacatagcagtggtgttacccgtgaactcatgcgtgagcttaacggaggggcatacactcgctatgtcgataacaacttctgtggccctgatggctaccctcttgagtgcattaaagaccttctagcacgtgctggtaaagcttcatgcactttgtccgaacaactggactttattgacactaagaggggtgtatactgctgccgtgaacatgagcatgaaattgcttggtacacggaacgttctgaaaagagctatgaattgcagacaccttttgaaattaaattggcaaagaaatttgacaccttcaatggggaatgtccaaattttgtatttcccttaaattccataatcaagactattcaaccaagggttgaaaagaaaaagcttgatggctttatgggtagaattcgatctgtctatccagttgcgtcaccaaatgaatgcaaccaaatgtgcctttcaactctcatgaagtgtgatcattgtggtgaaacttcatggcagacgggcgattttgttaaagccacttgcgaattttgtggcactgagaatttgactaaagaaggtgccactacttgtggttacttaccccaaaatgctgttgttaaaatttattgtccagcatgtcacaattcagaagtaggacctgagcatagtcttgccgaataccataatgaatctggcttgaaaaccattcttcgtaagggtggtcgcactattgcctttggaggctgtgtgttctcttatgttggttgccataacaagtgtgcctattgggttccacgtgctagcgctaacataggttgtaaccatacaggtgttgttggagaaggttccgaaggtcttaatgacaaccttcttgaaatactccaaaaagagaaagtcaacatcaatattgttggtgactttaaacttaatgaagagatcgccattattttggcatctttttctgcttccacaagtgcttttgtggaaactgtgaaaggtttggattataaagcattcaaacaaattgttgaatcctgtggtaattttaaagttacaaaaggaaaagctaaaaaaggtgcctggaatattggtgaacagaaatcaatactgagtcctctttatgcatttgcatcagaggctgctcgtgttgtacgatcaattttctcccgcactcttgaaactgctcaaaattctgtgcgtgttttacagaaggccgctataacaatactagatggaatttcacagtattcactgagactcattgatgctatgatgttcacatctgatttggctactaacaatctagttgtaatggcctacattacaggtggtgttgttcagttgacttcgcagtggctaactaacatctttggcactgtttatgaaaaactcaaacccgtccttgattggcttgaagagaagtttaaggaaggtgtagagtttcttagagacggttgggaaattgttaaatttatctcaacctgtgcttgtgaaattgtcggtggacaaattgtcacctgtgcaaaggaaattaaggagagtgttcagacattctttaagcttgtaaataaatttttggctttgtgtgctgactctatcattattggtggagctaaacttaaagccttgaatttaggtgaaacatttgtcacgcactcaaagggattgtacagaaagtgtgttaaatccagagaagaaactggcctactcatgcctctaaaagccccaaaagaaattatcttcttagagggagaaacacttcccacagaagtgttaacagaggaagttgtcttgaaaactggtgatttacaaccattagaacaacctactagtgaagctgttgaagctccattggttggtacaccagtttgtattaacgggcttatgttgctcgaaatcaaagacacagaaaagtactgtgcccttgcacctaatatgatggtaacaaacaataccttcacactcaaaggcggtgcaccaacaaaggttacttttggtgatgacactgtgatagaagtgcaaggttacaagagtgtgaatatcacttttgaacttgatgaaaggattgataaagtacttaatgagaagtgctctgcctatacagttgaactcggtacagaagtaaatgagttcgcctgtgttgtggcagatgctgtcataaaaactttgcaaccagtatctgaattacttacaccactgggcattgatttagatgagtggagtatggctacatactacttatttgatgagtctggtgagtttaaattggcttcacatatgtattgttctttctaccctccagatgaggatgaagaagaaggtgattgtgaagaagaagagtttgagccatcaactcaatatgagtatggtactgaagatgattaccaaggtaaacctttggaatttggtgccacttctgctgctcttcaacctgaagaagagcaagaagaagattggttagatgatgatagtcaacaaactgttggtcaacaagacggcagtgaggacaatcagacaactactattcaaacaattgttgaggttcaacctcaattagagatggaacttacaccagttgttcagactattgaagtgaatagttttagtggttatttaaaacttactgacaatgtatacattaaaaatgcagacattgtggaagaagctaaaaaggtaaaaccaacagtggttgttaatgcagccaatgtttaccttaaacatggaggaggtgttgcaggagccttaaataaggctactaacaatgccatgcaagttgaatctgatgattacatagctactaatggaccacttaaagtgggtggtagttgtgttttaagcggacacaatcttgctaaacactgtcttcatgttgtcggcccaaatgttaacaaaggtgaagacattcaacttcttaagagtgcttatgaaaattttaatcagcacgaagttctacttgcaccattattatcagctggtatttttggtgctgaccctatacattctttaagagtttgtgtagatactgttcgcacaaatgtctacttagctgtctttgataaaaatctctatgacaaacttgtttcaagctttttggaaatgaagagtgaaaagcaagttgaacaaaagatcgctgagattcctaaagaggaagttaagccatttataactgaaagtaaaccttcagttgaacagagaaaacaagatgataagaaaatcaaagcttgtgttgaagaagttacaacaactctggaagaaactaagttcctcacagaaaacttgttactttatattgacattaatggcaatcttcatccagattctgccactcttgttagtgacattgacatcactttcttaaagaaagatgctccatatatagtgggtgatgttgttcaagagggtgttttaactgctgtggttatacctactaaaaaggctggtggcactactgaaatgctagcgaaagctttgagaaaagtgccaacagacaattatataaccacttacccgggtcagggtttaaatggttacactgtagaggaggcaaagacagtgcttaaaaagtgtaaaagtgccttttacattctaccatctattatctctaatgagaagcaagaaattcttggaactgtttcttggaatttgcgagaaatgcttgcacatgcagaagaaacacgcaaattaatgcctgtctgtgtggaaactaaagccatagtttcaactatacagcgtaaatataagggtattaaaatacaagagggtgtggttgattatggtgctagattttacttttacaccagtaaaacaactgtagcgtcacttatcaacacacttaacgatctaaatgaaactcttgttacaatgccacttggctatgtaacacatggcttaaatttggaagaagctgctcggtatatgagatctctcaaagtgccagctacagtttctgtttcttcacctgatgctgttacagcgtataatggttatcttacttcttcttctaaaacacctgaagaacattttattgaaaccatctcacttgctggttcctataaagattggtcctattctggacaatctacacaactaggtatagaatttcttaagagaggtgataaaagtgtatattacactagtaatcctaccacattccacctagatggtgaagttatcacctttgacaatcttaagacacttctttctttgagagaagtgaggactattaaggtgtttacaacagtagacaacattaacctccacacgcaagttgtggacatgtcaatgacatatggacaacagtttggtccaacttatttggatggagctgatgttactaaaataaaacctcataattcacatgaaggtaaaacattttatgttttacctaatgatgacactctacgtgttgaggcttttgagtactaccacacaactgatcctagttttctgggtaggtacatgtcagcattaaatcacactaaaaagtggaaatacccacaagttaatggtttaacttctattaaatgggcagataacaactgttatcttgccactgcattgttaacactccaacaaatagagttgaagtttaatccacctgctctacaagatgcttattacagagcaagggctggtgaagctgctaacttttgtgcacttatcttagcctactgtaataagacagtaggtgagttaggtgatgttagagaaacaatgagttacttgtttcaacatgccaatttagattcttgcaaaagagtcttgaacgtggtgtgtaaaacttgtggacaacagcagacaacccttaagggtgtagaagctgttatgtacatgggcacactttcttatgaacaatttaagaaaggtgttcagataccttgtacgtgtggtaaacaagctacaaaatatctagtacaacaggagtcaccttttgttatgatgtcagcaccacctgctcagtatgaacttaagcatggtacatttacttgtgctagtgagtacactggtaattaccagtgtggtcactataaacatataacttctaaagaaactttgtattgcatagacggtgctttacttacaaagtcctcagaatacaaaggtcctattacggatgttttctacaaagaaaacagttacacaacaaccataaaaccagttacttataaattggatggtgttgtttgtacagaaattgaccctaagttggacaattattataagaaagacaattcttatttcacagagcaaccaattgatcttgtaccaaaccaaccatatccaaacgcaagcttcgataattttaagtttgtatgtgataatatcaaatttgctgatgatttaaaccagttaactggttataagaaacctgcttcaagagagcttaaagttacatttttccctgacttaaatggtgatgtggtggctattgattataaacactacacaccctcttttaagaaaggagctaaattgttacataaacctattgtttggcatgttaacaatgcaactaataaagccacgtataaaccaaatacctggtgtatacgttgtctttggagcacaaaaccagttgaaacatcaaattcgtttgatgtactgaagtcagaggacgcgcagggaatggataatcttgcctgcgaagatctaaaaccagtctctgaagaagtagtggaaaatcctaccatacagaaagacgttcttgagtgtaatgtgaaaactaccgaagttgtaggagacattatacttaaaccagcaaataatagtttaaaaattacagaagaggttggccacacagatctaatggctgcttatgtagacaattctagtcttactattaagaaacctaatgaattatctagagtattaggtttgaaaacccttgctactcatggtttagctgctgttaatagtgtcccttgggatactatagctaattatgctaagccttttcttaacaaagttgttagtacaactactaacatagttacacggtgtttaaaccgtgtttgtactaattatatgccttatttctttactttattgctacaattgtgtacttttactagaagtacaaattctagaattaaagcatctatgccgactactatagcaaagaatactgttaagagtgtcggtaaattttgtctagaggcttcatttaattatttgaagtcacctaatttttctaaactgataaatattataatttggtttttactattaagtgtttgcctaggttctttaatctactcaaccgctgctttaggtgttttaatgtctaatttaggcatgccttcttactgtactggttacagagaaggctatttgaactctactaatgtcactattgcaacctactgtactggttctataccttgtagtgtttgtcttagtggtttagattctttagacacctatccttctttagaaactatacaaattaccatttcatcttttaaatgggatttaactgcttttggcttagttgcagagtggtttttggcatatattcttttcactaggtttttctatgtacttggattggctgcaatcatgcaattgtttttcagctattttgcagtacattttattagtaattcttggcttatgtggttaataattaatcttgtacaaatggccccgatttcagctatggttagaatgtacatcttctttgcatcattttattatgtatggaaaagttatgtgcatgttgtagacggttgtaattcatcaacttgtatgatgtgttacaaacgtaatagagcaacaagagtcgaatgtacaactattgttaatggtgttagaaggtccttttatgtctatgctaatggaggtaaaggcttttgcaaactacacaattggaattgtgttaattgtgatacattctgtgctggtagtacatttattagtgatgaagttgcgagagacttgtcactacagtttaaaagaccaataaatcctactgaccagtcttcttacatcgttgatagtgttacagtgaagaatggttccatccatctttactttgataaagctggtcaaaagacttatgaaagacattctctctctcattttgttaacttagacaacctgagagctaataacactaaaggttcattgcctattaatgttatagtttttgatggtaaatcaaaatgtgaagaatcatctgcaaaatcagcgtctgtttactacagtcagcttatgtgtcaacctatactgttactagatcaggcattagtgtctgatgttggtgatagtgcggaagttgcagttaaaatgtttgatgcttacgttaatacgttttcatcaacttttaacgtaccaatggaaaaactcaaaacactagttgcaactgcagaagctgaacttgcaaagaatgtgtccttagacaatgtcttatctacttttatttcagcagctcggcaagggtttgttgattcagatgtagaaactaaagatgttgttgaatgtcttaaattgtcacatcaatctgacatagaagttactggcgatagttgtaataactatatgctcacctataacaaagttgaaaacatgacaccccgtgaccttggtgcttgtattgactgtagtgcgcgtcatattaatgcgcaggtagcaaaaagtcacaacattgctttgatatggaacgttaaagatttcatgtcattgtctgaacaactacgaaaacaaatacgtagtgctgctaaaaagaataacttaccttttaagttgacatgtgcaactactagacaagttgttaatgttgtaacaacaaagatagcacttaagggtggtaaaattgttaataattggttgaagcagttaattaaagttacacttgtgttcctttttgttgctgctattttctatttaataacacctgttcatgtcatgtctaaacatactgacttttcaagtgaaatcataggatacaaggctattgatggtggtgtcactcgtgacatagcatctacagatacttgttttgctaacaaacatgctgattttgacacatggtttagccagcgtggtggtagttatactaatgacaaagcttgcccattgattgctgcagtcataacaagagaagtgggttttgtcgtgcctggtttgcctggcacgatattacgcacaactaatggtgactttttgcatttcttacctagagtttttagtgcagttggtaacatctgttacacaccatcaaaacttatagagtacactgactttgcaacatcagcttgtgttttggctgctgaatgtacaatttttaaagatgcttctggtaagccagtaccatattgttatgataccaatgtactagaaggttctgttgcttatgaaagtttacgccctgacacacgttatgtgctcatggatggctctattattcaatttcctaacacctaccttgaaggttctgttagagtggtaacaacttttgattctgagtactgtaggcacggcacttgtgaaagatcagaagctggtgtttgtgtatctactagtggtagatgggtacttaacaatgattattacagatctttaccaggagttttctgtggtgtagatgctgtaaatttacttactaatatgtttacaccactaattcaacctattggtgctttggacatatcagcatctatagtagctggtggtattgtagctatcgtagtaacatgccttgcctactattttatgaggtttagaagagcttttggtgaatacagtcatgtagttgcctttaatactttactattccttatgtcattcactgtactctgtttaacaccagtttactcattcttacctggtgtttattctgttatttacttgtacttgacattttatcttactaatgatgtttcttttttagcacatattcagtggatggttatgttcacacctttagtacctttctggataacaattgcttatatcatttgtatttccacaaagcatttctattggttctttagtaattacctaaagagacgtgtagtctttaatggtgtttcctttagtacttttgaagaagctgcgctgtgcacctttttgttaaataaagaaatgtatctaaagttgcgtagtgatgtgctattacctcttacgcaatataatagatacttagctctttataataagtacaagtattttagtggagcaatggatacaactagctacagagaagctgcttgttgtcatctcgcaaaggctctcaatgacttcagtaactcaggttctgatgttctttaccaaccaccacaaacctctatcacctcagctgttttgcagagtggttttagaaaaatggcattcccatctggtaaagttgagggttgtatggtacaagtaacttgtggtacaactacacttaacggtctttggcttgatgacgtagtttactgtccaagacatgtgatctgcacctctgaagacatgcttaaccctaattatgaagatttactcattcgtaagtctaatcataatttcttggtacaggctggtaatgttcaactcagggttattggacattctatgcaaaattgtgtacttaagcttaaggttgatacagccaatcctaagacacctaagtataagtttgttcgcattcaaccaggacagactttttcagtgttagcttgttacaatggttcaccatctggtgtttaccaatgtgctatgaggcccaatttcactattaagggttcattccttaatggttcatgtggtagtgttggttttaacatagattatgactgtgtctctttttgttacatgcaccatatggaattaccaactggagttcatgctggcacagacttagaaggtaacttttatggaccttttgttgacaggcaaacagcacaagcagctggtacggacacaactattacagttaatgttttagcttggttgtacgctgctgttataaatggagacaggtggtttctcaatcgatttaccacaactcttaatgactttaaccttgtggctatgaagtacaattatgaacctctaacacaagaccatgttgacatactaggacctctttctgctcaaactggaattgccgttttagatatgtgtgcttcattaaaagaattactgcaaaatggtatgaatggacgtaccatattgggtagtgctttattagaagatgaatttacaccttttgatgttgttagacaatgctcaggtgttactttccaaagtgcagtgaaaagaacaatcaagggtacacaccactggttgttactcacaattttgacttcacttttagttttagtccagagtactcaatggtctttgttcttttttttgtatgaaaatgcctttttaccttttgctatgggtattattgctatgtctgcttttgcaatgatgtttgtcaaacataagcatgcatttctctgtttgtttttgttaccttctcttgccactgtagcttattttaatatggtctatatgcctgctagttgggtgatgcgtattatgacatggttggatatggttgatactagtttgtctggttttaagctaaaagactgtgttatgtatgcatcagctgtagtgttactaatccttatgacagcaagaactgtgtatgatgatggtgctaggagagtgtggacacttatgaatgtcttgacactcgtttataaagtttattatggtaatgctttagatcaagccatttccatgtgggctcttataatctctgttacttctaactactcaggtgtagttacaactgtcatgtttttggccagaggtattgtttttatgtgtgttgagtattgccctattttcttcataactggtaatacacttcagtgtataatgctagtttattgtttcttaggctatttttgtacttgttactttggcctcttttgtttactcaaccgctactttagactgactcttggtgtttatgattacttagtttctacacaggagtttagatatatgaattcacagggactactcccacccaagaatagcatagatgccttcaaactcaacattaaattgttgggtgttggtggcaaaccttgtatcaaagtagccactgtacagtctaaaatgtcagatgtaaagtgcacatcagtagtcttactctcagttttgcaacaactcagagtagaatcatcatctaaattgtgggctcaatgtgtccagttacacaatgacattctcttagctaaagatactactgaagcctttgaaaaaatggtttcactactttctgttttgctttccatgcagggtgctgtagacataaacaagctttgtgaagaaatgctggacaacagggcaaccttacaagctatagcctcagagtttagttcccttccatcatatgcagcttttgctactgctcaagaagcttatgagcaggctgttgctaatggtgattctgaagttgttcttaaaaagttgaagaagtctttgaatgtggctaaatctgaatttgaccgtgatgcagccatgcaacgtaagttggaaaagatggctgatcaagctatgacccaaatgtataaacaggctagatctgaggacaagagggcaaaagttactagtgctatgcagacaatgcttttcactatgcttagaaagttggataatgatgcactcaacaacattatcaacaatgcaagagatggttgtgttcccttgaacataatacctcttacaacagcagccaaactaatggttgtcataccagactataacacatataaaaatacgtgtgatggtacaacatttacttatgcatcagcattgtgggaaatccaacaggttgtagatgcagatagtaaaattgttcaacttagtgaaattagtatggacaattcacctaatttagcatggcctcttattgtaacagctttaagggccaattctgctgtcaaattacagaataatgagcttagtcctgttgcactacgacagatgtcttgtgctgccggtactacacaaactgcttgcactgatgacaatgcgttagcttactacaacacaacaaagggaggtaggtttgtacttgcactgttatccgatttacaggatttgaaatgggctagattccctaagagtgatggaactggtactatctatacagaactggaaccaccttgtaggtttgttacagacacacctaaaggtcctaaagtgaagtatttatactttattaaaggattaaacaacctaaatagaggtatggtacttggtagtttagctgccacagtacgtctacaagctggtaatgcaacagaagtgcctgccaattcaactgtattatctttctgtgcttttgctgtagatgctgctaaagcttacaaagattatctagctagtgggggacaaccaatcactaattgtgttaagatgttgtgtacacacactggtactggtcaggcaataacagttacaccggaagccaatatggatcaagaatcctttggtggtgcatcgtgttgtctgtactgccgttgccacatagatcatccaaatcctaaaggattttgtgacttaaaaggtaagtatgtacaaatacctacaacttgtgctaatgaccctgtgggttttacacttaaaaacacagtctgtaccgtctgcggtatgtggaaaggttatggctgtagttgtgatcaactccgcgaacccatgcttcagtcagctgatgcacaatcgtttttaaacgggtttgcggtgtaagtgcagcccgtcttacaccgtgcggcacaggcactagtactgatgtcgtatacagggcttttgacatctacaatgataaagtagctggttttgctaaattcctaaaaactaattgttgtcgcttccaagaaaaggacgaagatgacaatttaattgattcttactttgtagttaagagacacactttctctaactaccaacatgaagaaacaatttataatttacttaaggattgtccagctgttgctaaacatgacttctttaagtttagaatagacggtgacatggtaccacatatatcacgtcaacgtcttactaaatacacaatggcagacctcgtctatgctttaaggcattttgatgaaggtaattgtgacacattaaaagaaatacttgtcacatacaattgttgtgatgatgattatttcaataaaaaggactggtatgattttgtagaaaacccagatatattacgcgtatacgccaacttaggtgaacgtgtacgccaagctttgttaaaaacagtacaattctgtgatgccatgcgaaatgctggtattgttggtgtactgacattagataatcaagatctcaatggtaactggtatgatttcggtgatttcatacaaaccacgccaggtagtggagttcctgttgtagattcttattattcattgttaatgcctatattaaccttgaccagggctttaactgcagagtcacatgttgacactgacttaacaaagccttacattaagtgggatttgttaaaatatgacttcacggaagagaggttaaaactctttgaccgttattttaaatattgggatcagacataccacccaaattgtgttaactgtttggatgacagatgcattctgcattgtgcaaactttaatgttttattctctacagtgttcccacctacaagttttggaccactagtgagaaaaatatttgttgatggtgttccatttgtagtttcaactggataccacttcagagagctaggtgttgtacataatcaggatgtaaacttacatagctctagacttagttttaaggaattacttgtgtatgctgctgaccctgctatgcacgctgcttctggtaatctattactagataaacgcactacgtgcttttcagtagctgcacttactaacaatgttgcttttcaaactgtcaaacccggtaattttaacaaagacttctatgactttgctgtgtctaagggtttctttaaggaaggaagttctgttgaattaaaacacttcttctttgctcaggatggtaatgctgctatcagcgattatgactactatcgttataatctaccaacaatgtgtgatatcagacaactactatttgtagttgaagttgttgataagtactttgattgttacgatggtggctgtattaatgctaaccaagtcatcgtcaacaacctagacaaatcagctggttttccatttaataaatggggtaaggctagactttattatgattcaatgagttatgaggatcaagatgcacttttcgcatatacaaaacgtaatgtcatccctactataactcaaatgaatcttaagtatgccattagtgcaaagaatagagctcgcaccgtagctggtgtctctatctgtagtactatgaccaatagacagtttcatcaaaaattattgaaatcaatagccgccactagaggagctactgtagtaattggaacaagcaaattctatggtggttggcacaacatgttaaaaactgtttatagtgatgtagaaaaccctcaccttatgggttgggattatcctaaatgtgatagagccatgcctaacatgcttagaattatggcctcacttgttcttgctcgcaaacatacaacgtgttgtagcttgtcacaccgtttctatagattagctaatgagtgtgctcaagtattgagtgaaatggtcatgtgtggcggttcactatatgttaaaccaggtggaacctcatcaggagatgccacaactgcttatgctaatagtgtttttaacatttgtcaagctgtcacggccaatgttaatgcacttttatctactgatggtaacaaaattgccgataagtatgtccgcaatttacaacacagactttatgagtgtctctatagaaatagagatgttgacacagactttgtgaatgagttttacgcatatttgcgtaaacatttctcaatgatgatactctctgacgatgctgttgtgtgtttcaatagcacttatgcatctcaaggtctagtggctagcataaagaactttaagtcagttctttattatcaaaacaatgtttttatgtctgaagcaaaatgttggactgagactgaccttactaaaggacctcatgaattttgctctcaacatacaatgctagttaaacagggtgatgattatgtgtaccttccttacccagatccatcaagaatcctaggggccggctgttttgtagatgatatcgtaaaaacagatggtacacttatgattgaacggttcgtgtctttagctatagatgcttacccacttactaaacatcctaatcaggagtatgctgatgtctttcatttgtacttacaatacataagaaagctacatgatgagttaacaggacacatgttagacatgtattctgttatgcttactaatgataacacttcaaggtattgggaacctgagttttatgaggctatgtacacaccgcatacagtcttacaggctgttggggcttgtgttctttgcaattcacagacttcattaagatgtggtgcttgcatacgtagaccattcttatgttgtaaatgctgttacgaccatgtcatatcaacatcacataaattagtcttgtctgttaatccgtatgtttgcaatgctccaggttgtgatgtcacagatgtgactcaactttacttaggaggtatgagctattattgtaaatcacataaaccacccattagttttccattgtgtgctaatggacaagtttttggtttatataaaaatacatgtgttggtagcgataatgttactgactttaatgcaattgcaacatgtgactggacaaatgctggtgattacattttagctaacacctgtactgaaagactcaagctttttgcagcagaaacgctcaaagctactgaggagacatttaaactgtcttatggtattgctactgtacgtgaagtgctgtctgacagagaattacatctttcatgggaagttggtaaacctagaccaccacttaaccgaaattatgtctttactggttatcgtgtaactaaaaacagtaaagtacaaataggagagtacacctttgaaaaaggtgactatggtgatgctgttgtttaccgaggtacaacaacttacaaattaaatgttggtgattattttgtgctgacatcacatacagtaatgccattaagtgcacctacactagtgccacaagagcactatgttagaattactggcttatacccaacactcaatatctcagatgagttttctagcaatgttgcaaattatcaaaaggttggtatgcaaaagtattctacactccagggaccacctggtactggtaagagtcattttgctattggcctagctctctactacccttctgctcgcatagtgtatacagcttgctctcatgccgctgttgatgcactatgtgagaaggcattaaaatatttgcctatagataaatgtagtagaattatacctgcacgtgctcgtgtagagtgttttgataaattcaaagtgaattcaacattagaacagtatgtcttttgtactgtaaatgcattgcctgagacgacagcagatatagttgtctttgatgaaatttcaatggccacaaattatgatttgagtgttgtcaatgccagattacgtgctaagcactatgtgtacattggcgaccctgctcaattacctgcaccacgcacattgctaactaagggcacactagaaccagaatatttcaattcagtgtgtagacttatgaaaactataggtccagacatgttcctcggaacttgtcggcgttgtcctgctgaaattgttgacactgtgagtgctttggtttatgataataagcttaaagcacataaagacaaatcagctcaatgctttaaaatgttttataagggtgttatcacgcatgatgtttcatctgcaattaacaggccacaaataggcgtggtaagagaattccttacacgtaaccctgcttggagaaaagctgtctttatttcaccttataattcacagaatgctgtagcctcaaagattttgggactaccaactcaaactgttgattcatcacagggctcagaatatgactatgtcatattcactcaaaccactgaaacagctcactcttgtaatgtaaacagatttaatgttgctattaccagagcaaaagtaggcatactttgcataatgtctgatagagacctttatgacaagttgcaatttacaagtcttgaaattccacgtaggaatgtggcaactttacaagctgaaaatgtaacaggactctttaaagattgtagtaaggtaatcactgggttacatcctacacaggcacctacacacctcagtgttgacactaaattcaaaactgaaggtttatgtgttgacatacctggcatacctaaggacatgacctatagaagactcatctctatgatgggttttaaaatgaattatcaagttaatggttaccctaacatgtttatcacccgcgaagaagctataagacatgtacgtgcatggattggcttcgatgtcgaggggtgtcatgctactagagaagctgttggtaccaatttacctttacagctaggtttttctacaggtgttaacctagttgctgtacctacaggttatgttgatacacctaataatacagatttttccagagttagtgctaaaccaccgcctggagatcaatttaaacacctcataccacttatgtacaaaggacttccttggaatgtagtgcgtataaagattgtacaaatgttaagtgacacacttaaaaatctctctgacagagtcgtatttgtcttatgggcacatggctttgagttgacatctatgaagtattttgtgaaaataggacctgagcgcacctgttgtctatgtgatagacgtgccacatgcttttccactgcttcagacacttatgcctgttggcatcattctattggatttgattacgtctataatccgtttatgattgatgttcaacaatggggttttacaggtaacctacaaagcaaccatgatctgtattgtcaagtccatggtaatgcacatgtagctagttgtgatgcaatcatgactaggtgtctagctgtccacgagtgctttgttaagcgtgttgactggactattgaatatcctataattggtgatgaactgaagattaatgcggcttgtagaaaggttcaacacatggttgttaaagctgcattattagcagacaaattcccagttcttcacgacattggtaaccctaaagctattaagtgtgtacctcaagctgatgtagaatggaagttctatgatgcacagccttgtagtgacaaagcttataaaatagaagaattattctattcttatgccacacattctgacaaattcacagatggtgtatgcctattttggaattgcaatgtcgatagatatcctgctaattccattgtttgtagatttgacactagagtgctatctaaccttaacttgcctggttgtgatggtggcagtttgtatgtaaataaacatgcattccacacaccagcttttgataaaagtgcttttgttaatttaaaacaattaccatttttctattactctgacagtccatgtgagtctcatggaaaacaagtagtgtcagatatagattatgtaccactaaagtctgctacgtgtataacacgttgcaatttaggtggtgctgtctgtagacatcatgctaatgagtacagattgtatctcgatgcttataacatgatgatctcagctggctttagcttgtgggtttacaaacaatttgatacttataacctctggaacacttttacaagacttcagagtttagaaaatgtggcttttaatgttgtaaataagggacactttgatggacaacagggtgaagtaccagtttctatcattaataacactgtttacacaaaagttgatggtgttgatgtagaattgtttgaaaataaaacaacattacctgttaatgtagcatttgagctttgggctaagcgcaacattaaaccagtaccagaggtgaaaatactcaataatttgggtgtggacattgctgctaatactgtgatctgggactacaaaagagatgctccagcacatatatctactattggtgtttgttctatgactgacatagccaagaaaccaactgaaacgatttgtgcaccactcactgtcttttttgatggtagagttgatggtcaagtagacttatttagaaatgcccgtaatggtgttcttattacagaaggtagtgttaaaggtttacaaccatctgtaggtcccaaacaagctagtcttaatggagtcacattaattggagaagccgtaaaaacacagttcaattattataagaaagttgatggtgttgtccaacaattacctgaaacttactttactcagagtagaaatttacaagaatttaaacccaggagtcaaatggaaattgatttcttagaattagctatggatgaattcattgaacggtataaattagaaggctatgccttcgaacatatcgtttatggagattttagtcatagtcagttaggtggtttacatctactgattggactagctaaacgttttaaggaatcaccttttgaattagaagattttattcctatggacagtacagttaaaaactatttcataacagatgcgcaaacaggttcatctaagtgtgtgtgttctgttattgatttattacttgatgattttgttgaaataataaaatcccaagatttatctgtagtttctaaggttgtcaaagtgactattgactatacagaaatttcatttatgctttggtgtaaagatggccatgtagaaacattttacccaaaattacaatctagtcaagcgtggcaaccgggtgttgctatgcctaatctttacaaaatgcaaagaatgctattagaaaagtgtgaccttcaaaattatggtgatagtgcaacattacctaaaggcataatgatgaatgtcgcaaaatatactcaactgtgtcaatatttaaacacattaacattagctgtaccctataatatgagagttatacattttggtgctggttctgataaaggagttgcaccaggtacagctgttttaagacagtggttgcctacgggtacgctgcttgtcgattcagatcttaatgactttgtctctgatgcagattcaactttgattggtgattgtgcaactgtacatacagctaataaatgggatctcattattagtgatatgtacgaccctaagactaaaaatgttacaaaagaaaatgactctaaagagggttttttcacttacatttgtgggtttatacaacaaaagctagctcttggaggttccgtggctataaagataacagaacattcttggaatgctgatctttataagctcatgggacacttcgcatggtggacagcctttgttactaatgtgaatgcgtcatcatctgaagcatttttaattggatgtaattatcttggcaaaccacgcgaacaaatagatggttatgtcatgcatgcaaattacatattttggaggaatacaaatccaattcagttgtcttcctattctttatttgacatgagtaaatttccccttaaattaaggggtactgctgttatgtctttaaaagaaggtcaaatcaatgatatgattttatctcttcttagtaaaggtagacttataattagagaaaacaacagagttgttatttctagtgatgttcttgttaacaactaa